European Patent Specification EP 3 856 154 B1, published August 27, 2025. Title: IMPLANTABLE DEVICES FOR CELL THERAPY AND RELATED METHODS. Applicant: SIGILON THERAPEUTICS, INC. The sequence listing filed with the application follows.

SEQUENCE LISTING (70 sequences)

SEQ ID NO: 1 - protein, 1457 aa, Artificial Sequence
  source: /note="Description of Artificial Sequence: Synthetic polypeptide"
MQIELSTCFFLCLLRFCFSATRRYYLGAVELSWDYMQSDLGELPVDARFPPRVPKSFPFNTSVVYKKTLFVEFTDHLFNIAKPRPPWMGLLGPTIQAEVYDTVVITLKNMASHPVSLHAVGVSYWKASEGAEYDDQTSQREKEDDKVFPGGSHTYVWQVLKENGPMASDPLCLTYSYLSHVDLVKDLNSGLIGALLVCREGSLAKEKTQTLHKFILLFAVFDEGKSWHSETKNSLMQDRDAASARAWPKMHTVNGYVNRSLPGLIGCHRKSVYWHVIGMGTTPEVHSIFLEGHTFLVRNHRQASLEISPITFLTAQTLLMDLGQFLLFCHISSHQHDGMEAYVKVDSCPEEPQLRMKNNEEAEDYDDDLTDSEMDVVRFDDDNSPSFIQIRSVAKKHPKTWVHYIAAEEEDWDYAPLVLAPDDRSYKSQYLNNGPQRIGRKYKKVRFMAYTDETFKTREAIQHESGILGPLLYGEVGDTLLIIFKNQASRPYNIYPHGITDVRPLYSRRLPKGVKHLKDFPILPGEIFKYKWTVTVEDGPTKSDPRCLTRYYSSFVNMERDLASGLIGPLLICYKESVDQRGNQIMSDKRNVILFSVFDENRSWYLTENIQRFLPNPAGVQLEDPEFQASNIMHSINGYVFDSLQLSVCLHEVAYWYILSIGAQTDFLSVFFSGYTFKHKMVYEDTLTLFPFSGETVFMSMENPGLWILGCHNSDFRNRGMTALLKVSSCDKNTGDYYEDSYEDISAYLLSKNNAIEPRSFSQNPPVLKRHQREITRTTLQSDQEEIDYDDTISVEMKKEDFDIYDEDENQSPRSFQKKTRHYFIAAVERLWDYGMSSSPHVLRNRAQSGSVPQFKKVVFQEFTDGSFTQPLYRGELNEHLGLLGPYIRAEVEDNIMVTFRNQASRPYSFYSSLISYEEDQRQGAEPRKNFVKPNETKTYFWKVQHHMAPTKDEFDCKAWAYFSDVDLEKDVHSGLIGPLLVCHTNTLNPAHGRQVTVQEFALFFTIFDETKSWYFTENMERNCRAPCNIQMEDPTFKENYRFHAINGYIMDTLPGLVMAQDQRIRWYLLSMGSNENIHSIHFSGHVFTVRKKEEYKMALYNLYPGVFETVEMLPSKAGIWRVECLIGEHLHAGMSTLFLVYSNKCQTPLGMASGHIRDFQITASGQYGQWAPKLARLHYSGSINAWSTKEPFSWIKVDLLAPMIIHGIKTQGARQKFSSLYISQFIIMYSLDGKKWQTYRGNSTGTLMVFFGNVDSSGIKHNIFNPPIIARYIRLHPTHYSIRSTLRMELMGCDLNSCSMPLGMESKAISDAQITASSYFTNMFATWSPSKARLHLQGRSNAWRPQVNNPKEWLQVDFQKTMKVTGVTTQGVKSLLTSMYVKEFLISSSQDGHQWTLFFQNGKVKVFQGNQDSFTPVVNSLDPPLLTRYLRIHPQSWVHQIALRMEVLGCEAQDLY

SEQ ID NO: 2 - protein, 415 aa, Artificial Sequence
  source: /note="Description of Artificial Sequence: Synthetic polypeptide"
YNSGKLEEFVQGNLERECMEEKCSFEEAREVFENTERTTEFWKQYVDGDQCESNPCLNGGSCKDDINSYECWCPFGFEGKNCELDVTCNIKNGRCEQFCKNSADNKVVCSCTEGYRLAENQKSCEPAVPFPCGRVSVSQTSKLTRAETVFPDVDYVNSTEAETILDNITQSTQSFNDFTRVVGGEDAKPGQFPWQVVLNGKVDAFCGGSIVNEKWIVTAAHCVETGVKITVVAGEHNIEETEHTEQKRNVIRIIPHHNYNAAINKYNHDIALLELDEPLVLNSYVTPICIADKEYTNIFLKFGSGYVSGWGRVFHKGRSALVLQYLRVPLVDRATCLRSTKFTIYNNMFCAGFHEGGRDSCQGDSGGPHVTEVEGTSFLTGIISWGEECAMKGKYGIYTKVSRYVNWIKEKTKLT

SEQ ID NO: 3 - protein, 1457 aa, Artificial Sequence
  source: /note="Description of Artificial Sequence: Synthetic polypeptide"
MQIELSTCFFLCLLRFCFSATRRYYLGAVELSWDYMQSDLGELPVDARFPPRVPKSFPFNTSVVYKKTLFVEFTDHLFNIAKPRPPWMGLLGPTIQAEVYDTVVITLKNMASHPVSLHAVGVSYWKASEGAEYDDQTSQREKEDDKVFPGGSHTYVWQVLKENGPMASDPLCLTYSYLSHVDLVKDLNSGLIGALLVCREGSLAKEKTQTLHKFILLFAVFDEGKSWHSETKNSLMQDRDAASARAWPKMHTVNGYVNRSLPGLIGCHRKSVYWHVIGMGTTPEVHSIFLEGHTFLVRNHRQASLEISPITFLTAQTLLMDLGQFLLFCHISSHQHDGMEAYVKVDSCPEEPQLRMKNNEEAEDYDDDLTDSEMDVVRFDDDNSPSFIQIRSVAKKHPKTWVHYIAAEEEDWDYAPLVLAPDDRSYKSQYLNNGPQRIGRKYKKVRFMAYTDETFKTREAIQHESGILGPLLYGEVGDTLLIIFKNQASRPYNIYPHGITDVRPLYSRRLPKGVKHLKDFPILPGEIFKYKWTVTVEDGPTKSDPRCLTRYYSSFVNMERDLASGLIGPLLICYKESVDQRGNQIMSDKRNVILFSVFDENRSWYLTENIQRFLPNPAGVQLEDPEFQASNIMHSINGYVFDSLQLSVCLHEVAYWYILSIGAQTDFLSVFFSGYTFKHKMVYEDTLTLFPFSGETVFMSMENPGLWILGCHNSDFRNRGMTALLKVSSCDKNTGDYYEDSYEDISAYLLSKNNAIEPRSFSQNPPVLKHHQREITRTTLQSDQEEIDYDDTISVEMKKEDFDIYDEDENQSPRSFQKKTRHYFIAAVERLWDYGMSSSPHVLRNRAQSGSVPQFKKVVFQEFTDGSFTQPLYRGELNEHLGLLGPYIRAEVEDNIMVTFRNQASRPYSFYSSLISYEEDQRQGAEPRKNFVKPNETKTYFWKVQHHMAPTKDEFDCKAWAYFSDVDLEKDVHSGLIGPLLVCHTNTLNPAHGRQVTVQEFALFFTIFDETKSWYFTENMERNCRAPCNIQMEDPTFKENYRFHAINGYIMDTLPGLVMAQDQRIRWYLLSMGSNENIHSIHFSGHVFTVRKKEEYKMALYNLYPGVFETVEMLPSKAGIWRVECLIGEHLHAGMSTLFLVYSNKCQTPLGMASGHIRDFQITASGQYGQWAPKLARLHYSGSINAWSTKEPFSWIKVDLLAPMIIHGIKTQGARQKFSSLYISQFIIMYSLDGKKWQTYRGNSTGTLMVFFGNVDSSGIKHNIFNPPIIARYIRLHPTHYSIRSTLRMELMGCDLNSCSMPLGMESKAISDAQITASSYFTNMFATWSPSKARLHLQGRSNAWRPQVNNPKEWLQVDFQKTMKVTGVTTQGVKSLLTSMYVKEFLISSSQDGHQWTLFFQNGKVKVFQGNQDSFTPVVNSLDPPLLTRYLRIHPQSWVHQIALRMEVLGCEAQDLY

SEQ ID NO: 4 - protein, 1457 aa, Artificial Sequence
  source: /note="Description of Artificial Sequence: Synthetic polypeptide"
MQIELSTCFFLCLLRFCFSATRRYYLGAVELSWDYMQSDLGELPVDARFPPRVPKSFPFNTSVVYKKTLFVEFTDHLFNIAKPRPPWMGLLGPTIQAEVYDTVVITLKNMASHPVSLHAVGVSYWKASEGAEYDDQTSQREKEDDKVFPGGSHTYVWQVLKENGPMASDPLCLTYSYLSHVDLVKDLNSGLIGALLVCREGSLAKEKTQTLHKFILLFAVFDEGKSWHSETKNSLMQDRDAASARAWPKMHTVNGYVNRSLPGLIGCHRKSVYWHVIGMGTTPEVHSIFLEGHTFLVRNHRQASLEISPITFLTAQTLLMDLGQFLLFCHISSHQHDGMEAYVKVDSCPEEPQLRMKNNEEAEDYDDDLTDSEMDVVRFDDDNSPSFIQIRSVAKKHPKTWVHYIAAEEEDWDYAPLVLAPDDRSYKSQYLNNGPQRIGRKYKKVRFMAYTDETFKTREAIQHESGILGPLLYGEVGDTLLIIFKNQASRPYNIYPHGITDVRPLYSRRLPKGVKHLKDFPILPGEIFKYKWTVTVEDGPTKSDPRCLTRYYSSFVNMERDLASGLIGPLLICYKESVDQRGNQIMSDKRNVILFSVFDENRSWYLTENIQRFLPNPAGVQLEDPEFQASNIMHSINGYVFDSLQLSVCLHEVAYWYILSIGAQTDFLSVFFSGYTFKHKMVYEDTLTLFPFSGETVFMSMENPGLWILGCHNSDFRNRGMTALLKVSSCDKNTGDYYEDSYEDISAYLLSKNNAIEPRSFSQNPPVLKAHQAEITRTTLQSDQEEIDYDDTISVEMKKEDFDIYDEDENQSPRSFQKKTRHYFIAAVERLWDYGMSSSPHVLRNRAQSGSVPQFKKVVFQEFTDGSFTQPLYRGELNEHLGLLGPYIRAEVEDNIMVTFRNQASRPYSFYSSLISYEEDQRQGAEPRKNFVKPNETKTYFWKVQHHMAPTKDEFDCKAWAYFSDVDLEKDVHSGLIGPLLVCHTNTLNPAHGRQVTVQEFALFFTIFDETKSWYFTENMERNCRAPCNIQMEDPTFKENYRFHAINGYIMDTLPGLVMAQDQRIRWYLLSMGSNENIHSIHFSGHVFTVRKKEEYKMALYNLYPGVFETVEMLPSKAGIWRVECLIGEHLHAGMSTLFLVYSNKCQTPLGMASGHIRDFQITASGQYGQWAPKLARLHYSGSINAWSTKEPFSWIKVDLLAPMIIHGIKTQGARQKFSSLYISQFIIMYSLDGKKWQTYRGNSTGTLMVFFGNVDSSGIKHNIFNPPIIARYIRLHPTHYSIRSTLRMELMGCDLNSCSMPLGMESKAISDAQITASSYFTNMFATWSPSKARLHLQGRSNAWRPQVNNPKEWLQVDFQKTMKVTGVTTQGVKSLLTSMYVKEFLISSSQDGHQWTLFFQNGKVKVFQGNQDSFTPVVNSLDPPLLTRYLRIHPQSWVHQIALRMEVLGCEAQDLY

SEQ ID NO: 5 - protein, 1453 aa, Artificial Sequence
  source: /note="Description of Artificial Sequence: Synthetic polypeptide"
MQIELSTCFFLCLLRFCFSATRRYYLGAVELSWDYMQSDLGELPVDARFPPRVPKSFPFNTSVVYKKTLFVEFTDHLFNIAKPRPPWMGLLGPTIQAEVYDTVVITLKNMASHPVSLHAVGVSYWKASEGAEYDDQTSQREKEDDKVFPGGSHTYVWQVLKENGPMASDPLCLTYSYLSHVDLVKDLNSGLIGALLVCREGSLAKEKTQTLHKFILLFAVFDEGKSWHSETKNSLMQDRDAASARAWPKMHTVNGYVNRSLPGLIGCHRKSVYWHVIGMGTTPEVHSIFLEGHTFLVRNHRQASLEISPITFLTAQTLLMDLGQFLLFCHISSHQHDGMEAYVKVDSCPEEPQLRMKNNEEAEDYDDDLTDSEMDVVRFDDDNSPSFIQIRSVAKKHPKTWVHYIAAEEEDWDYAPLVLAPDDRSYKSQYLNNGPQRIGRKYKKVRFMAYTDETFKTREAIQHESGILGPLLYGEVGDTLLIIFKNQASRPYNIYPHGITDVRPLYSRRLPKGVKHLKDFPILPGEIFKYKWTVTVEDGPTKSDPRCLTRYYSSFVNMERDLASGLIGPLLICYKESVDQRGNQIMSDKRNVILFSVFDENRSWYLTENIQRFLPNPAGVQLEDPEFQASNIMHSINGYVFDSLQLSVCLHEVAYWYILSIGAQTDFLSVFFSGYTFKHKMVYEDTLTLFPFSGETVFMSMENPGLWILGCHNSDFRNRGMTALLKVSSCDKNTGDYYEDSYEDISAYLLSKNNAIEPRSFSQNPPVLKEITRTTLQSDQEEIDYDDTISVEMKKEDFDIYDEDENQSPRSFQKKTRHYFIAAVERLWDYGMSSSPHVLRNRAQSGSVPQFKKVVFQEFTDGSFTQPLYRGELNEHLGLLGPYIRAEVEDNIMVTFRNQASRPYSFYSSLISYEEDQRQGAEPRKNFVKPNETKTYFWKVQHHMAPTKDEFDCKAWAYFSDVDLEKDVHSGLIGPLLVCHTNTLNPAHGRQVTVQEFALFFTIFDETKSWYFTENMERNCRAPCNIQMEDPTFKENYRFHAINGYIMDTLPGLVMAQDQRIRWYLLSMGSNENIHSIHFSGHVFTVRKKEEYKMALYNLYPGVFETVEMLPSKAGIWRVECLIGEHLHAGMSTLFLVYSNKCQTPLGMASGHIRDFQITASGQYGQWAPKLARLHYSGSINAWSTKEPFSWIKVDLLAPMIIHGIKTQGARQKFSSLYISQFIIMYSLDGKKWQTYRGNSTGTLMVFFGNVDSSGIKHNIFNPPIIARYIRLHPTHYSIRSTLRMELMGCDLNSCSMPLGMESKAISDAQITASSYFTNMFATWSPSKARLHLQGRSNAWRPQVNNPKEWLQVDFQKTMKVTGVTTQGVKSLLTSMYVKEFLISSSQDGHQWTLFFQNGKVKVFQGNQDSFTPVVNSLDPPLLTRYLRIHPQSWVHQIALRMEVLGCEAQDLY

SEQ ID NO: 6 - protein, 1454 aa, Artificial Sequence
  source: /note="Description of Artificial Sequence: Synthetic polypeptide"
MQIELSTCFFLCLLRFCFSATRRYYLGAVELSWDYMQSDLGELPVDARFPPRVPKSFPFNTSVVYKKTLFVEFTDHLFNIAKPRPPWMGLLGPTIQAEVYDTVVITLKNMASHPVSLHAVGVSYWKASEGAEYDDQTSQREKEDDKVFPGGSHTYVWQVLKENGPMASDPLCLTYSYLSHVDLVKDLNSGLIGALLVCREGSLAKEKTQTLHKFILLFAVFDEGKSWHSETKNSLMQDRDAASARAWPKMHTVNGYVNRSLPGLIGCHRKSVYWHVIGMGTTPEVHSIFLEGHTFLVRNHRQASLEISPITFLTAQTLLMDLGQFLLFCHISSHQHDGMEAYVKVDSCPEEPQLRMKNNEEAEDYDDDLTDSEMDVVRFDDDNSPSFIQIRSVAKKHPKTWVHYIAAEEEDWDYAPLVLAPDDRSYKSQYLNNGPQRIGRKYKKVRFMAYTDETFKTREAIQHESGILGPLLYGEVGDTLLIIFKNQASRPYNIYPHGITDVRPLYSRRLPKGVKHLKDFPILPGEIFKYKWTVTVEDGPTKSDPRCLTRYYSSFVNMERDLASGLIGPLLICYKESVDQRGNQIMSDKRNVILFSVFDENRSWYLTENIQRFLPNPAGVQLEDPEFQASNIMHSINGYVFDSLQLSVCLHEVAYWYILSIGAQTDFLSVFFSGYTFKHKMVYEDTLTLFPFSGETVFMSMENPGLWILGCHNSDFRNRGMTALLKVSSCDKNTGDYYEDSYEDISAYLLSKNNAIEPRSFSQNPPVLKREITRTTLQSDQEEIDYDDTISVEMKKEDFDIYDEDENQSPRSFQKKTRHYFIAAVERLWDYGMSSSPHVLRNRAQSGSVPQFKKVVFQEFTDGSFTQPLYRGELNEHLGLLGPYIRAEVEDNIMVTFRNQASRPYSFYSSLISYEEDQRQGAEPRKNFVKPNETKTYFWKVQHHMAPTKDEFDCKAWAYFSDVDLEKDVHSGLIGPLLVCHTNTLNPAHGRQVTVQEFALFFTIFDETKSWYFTENMERNCRAPCNIQMEDPTFKENYRFHAINGYIMDTLPGLVMAQDQRIRWYLLSMGSNENIHSIHFSGHVFTVRKKEEYKMALYNLYPGVFETVEMLPSKAGIWRVECLIGEHLHAGMSTLFLVYSNKCQTPLGMASGHIRDFQITASGQYGQWAPKLARLHYSGSINAWSTKEPFSWIKVDLLAPMIIHGIKTQGARQKFSSLYISQFIIMYSLDGKKWQTYRGNSTGTLMVFFGNVDSSGIKHNIFNPPIIARYIRLHPTHYSIRSTLRMELMGCDLNSCSMPLGMESKAISDAQITASSYFTNMFATWSPSKARLHLQGRSNAWRPQVNNPKEWLQVDFQKTMKVTGVTTQGVKSLLTSMYVKEFLISSSQDGHQWTLFFQNGKVKVFQGNQDSFTPVVNSLDPPLLTRYLRIHPQSWVHQIALRMEVLGCEAQDLY

SEQ ID NO: 7 - protein, 1474 aa, Artificial Sequence [sequence omitted]

SEQ ID NO: 8 - DNA, 4374 bp, Artificial Sequence
  source: /note="Description of Artificial Sequence: Synthetic polynucleotide"
atgcaaatagagctctccacctgcttctttctgtgccttttgcgattctgctttagtgccaccagaagatactacctgggtgcagtggaactgtcatgggactatatgcaaagtgatctcggtgagctgcctgtggacgcaagatttcctcctagagtgccaaaatcttttccattcaacacctcagtcgtgtacaaaaagactctgtttgtagaattcacggatcaccttttcaacatcgctaagccaaggccaccctggatgggtctgctaggtcctaccatccaggctgaggtttatgatacagtggtcattacacttaagaacatggcttcccatcctgtcagtcttcatgctgttggtgtatcctactggaaagcttctgagggagctgaatatgatgatcagaccagtcaaagggagaaagaagatgataaagtcttccctggtggaagccatacatatgtctggcaggtcctgaaagagaatggtccaatggcctctgacccactgtgccttacctactcatatctttctcatgtggacctggtaaaagacttgaattcaggcctcattggagccctactagtatgtagagaagggagtctggccaaggaaaagacacagaccttgcacaaatttatactactttttgctgtatttgatgaagggaaaagttggcactcagaaacaaagaactccttgatgcaggatagggatgctgcatctgctcgggcctggcctaaaatgcacacagtcaatggttatgtaaacaggtctctgccaggtctgattggatgccacaggaaatcagtctattggcatgtgattggaatgggcaccactcctgaagtgcactcaatattcctcgaaggtcacacatttcttgtgaggaaccatcgccaggcgtccttggaaatctcgccaataactttccttactgctcaaacactcttgatggaccttggacagtttctactgttttgtcatatctcttcccaccaacatgatggcatggaagcttatgtcaaagtagacagctgtccagaggaaccccaactacgaatgaaaaataatgaagaagcggaagactatgatgatgatcttactgattctgaaatggatgtggtcaggtttgatgatgacaactctccttcctttatccaaattcgctcagttgccaagaagcatcctaaaacttgggtacattacattgctgctgaagaggaggactgggactatgctcccttagtcctcgcccccgatgacagaagttataaaagtcaatatttgaacaatggccctcagcggattggtaggaagtacaaaaaagtccgatttatggcatacacagatgaaacctttaagactcgtgaagctattcagcatgaatcaggaatcttgggacctttactttatggggaagttggagacacactgttgattatatttaagaatcaagcaagcagaccatataacatctaccctcacggaatcactgatgtccgtcctttgtattcaaggagattaccaaaaggtgtaaaacatttgaaggattttccaattctgccaggagaaatattcaaatataaatggacagtgactgtagaagatgggccaactaaatcagatcctcggtgcctgacccgctattactctagtttcgttaatatggagagagatctagcttcaggactcattggccctctcctcatctgctacaaagaatctgtagatcaaagaggaaaccagataatgtcagacaagaggaatgtcatcctgttttctgtatttgatgagaaccgaagctggtacctcacagagaatatacaacgctttctccccaatccagctggagtgcagcttgaggatccagagttccaagcctccaacatcatgcacagcatcaatggctatgtttttgatagtttgcagttgtcagtttgtttgcatgaggtggcatactggtacattctaagcattggagcacagactgacttcctttctgtcttcttctctggatataccttcaaacacaaaatggtctatgaagacacactcaccctattcccattctcaggagaaactgtcttcatgtcgatggaaaacccaggtctatggattctggggtgccacaactcagactttcggaacagaggcatgaccgccttactgaaggtttctagttgtgacaagaacactggtgattattacgaggacagttatgaagatatttcagcatacttgctgagtaaaaacaatgccattgaaccaagaagcttctcccaaaacccaccagtcttgaaacgccatcaacgggaaataactcgtactactcttcagtcagatcaagaggaaattgactatgatgataccatatcagttgaaatgaagaaggaagattttgacatttatgatgaggatgaaaatcagagcccccgcagctttcaaaagaaaacacgacactattttattgctgcagtggagaggctctgggattatgggatgagtagctccccacatgttctaagaaacagggctcagagtggcagtgtccctcagttcaagaaagttgttttccaggaatttactgatggctcctttactcagcccttataccgtggagaactaaatgaacatttgggactcctggggccatatataagagcagaagttgaagataatatcatggtaactttcagaaatcaggcctctcgtccctattccttctattctagccttatttcttatgaggaagatcagaggcaaggagcagaacctagaaaaaactttgtcaagcctaatgaaaccaaaacttacttttggaaagtgcaacatcatatggcacccactaaagatgagtttgactgcaaagcctgggcttatttctctgatgttgacctggaaaaagatgtgcactcaggcctgattggaccccttctggtctgccacactaacacactgaaccctgctcatgggagacaagtgacagtacaggaatttgctctgtttttcaccatctttgatgagaccaaaagctggtacttcactgaaaatatggaaagaaactgcagggctccctgcaatatccagatggaagatcccacttttaaagagaattatcgcttccatgcaatcaatggctacataatggatacactacctggcttagtaatggctcaggatcaaaggattcgatggtatctgctcagcatgggcagcaatgaaaacatccattctattcatttcagtggacatgtgttcactgtacgaaaaaaagaggagtataaaatggcactgtacaatctctatccaggtgtttttgagacagtggaaatgttaccatccaaagctggaatttggcgggtggaatgccttattggcgagcatctacatgctgggatgagcacactttttctggtgtacagcaataagtgtcagactcccctgggaatggcttctggacacattagagattttcagattacagcttcaggacaatatggacagtgggccccaaagctggccagacttcattattccggatcaatcaatgcctggagcaccaaggagcccttttcttggatcaaggtggatctgttggcaccaatgattattcacggcatcaagacccagggtgcccgtcagaagttctccagcctctacatctctcagtttatcatcatgtatagtcttgatgggaagaagtggcagacttatcgaggaaattccactggaaccttaatggtcttctttggcaatgtggattcatctgggataaaacacaatatttttaaccctccaattattgctcgatacatccgtttgcacccaactcattatagcattcgcagcactcttcgcatggagttgatgggctgtgatttaaatagttgcagcatgccattgggaatggagagtaaagcaatatcagatgcacagattactgcttcatcctactttaccaatatgtttgccacctggtctccttcaaaagctcgacttcacctccaagggaggagtaatgcctggagacctcaggtgaataatccaaaagagtggctgcaagtggacttccagaagacaatgaaagtcacaggagtaactactcagggagtaaaatctctgcttaccagcatgtatgtgaaggagttcctcatctccagcagtcaagatggccatcagtggactctcttttttcagaatggcaaagtaaaggtttttcagggaaatcaagactccttcacacctgtggtgaactctctagacccaccgttactgactcgctaccttcgaattcacccccagagttgggtgcaccagattgccctgaggatggaggttctgggctgcgaggcacaggacctctactga

SEQ ID NO: 9 - DNA, 4374 bp, Artificial Sequence
  source: /note="Description of Artificial Sequence: Synthetic polynucleotide"
atgcaaatagagctctccacctgcttctttctgtgccttttgcgattctgctttagtgccaccagaagatactacctgggtgcagtggaactgtcatgggactatatgcaaagtgatctcggtgagctgcctgtggacgcaagatttcctcctagagtgccaaaatcttttccattcaacacctcagtcgtgtacaaaaagactctgtttgtagaattcacggatcaccttttcaacatcgctaagccaaggccaccctggatgggtctgctaggtcctaccatccaggctgaggtttatgatacagtggtcattacacttaagaacatggcttcccatcctgtcagtcttcatgctgttggtgtatcctactggaaagcttctgagggagctgaatatgatgatcagaccagtcaaagggagaaagaagatgataaagtcttccctggtggaagccatacatatgtctggcaggtcctgaaagagaatggtccaatggcctctgacccactgtgccttacctactcatatctttctcatgtggacctggtaaaagacttgaattcaggcctcattggagccctactagtatgtagagaagggagtctggccaaggaaaagacacagaccttgcacaaatttatactactttttgctgtatttgatgaagggaaaagttggcactcagaaacaaagaactccttgatgcaggatagggatgctgcatctgctcgggcctggcctaaaatgcacacagtcaatggttatgtaaacaggtctctgccaggtctgattggatgccacaggaaatcagtctattggcatgtgattggaatgggcaccactcctgaagtgcactcaatattcctcgaaggtcacacatttcttgtgaggaaccatcgccaggcgtccttggaaatctcgccaataactttccttactgctcaaacactcttgatggaccttggacagtttctactgttttgtcatatctcttcccaccaacatgatggcatggaagcttatgtcaaagtagacagctgtccagaggaaccccaactacgaatgaaaaataatgaagaagcggaagactatgatgatgatcttactgattctgaaatggatgtggtcaggtttgatgatgacaactctccttcctttatccaaattcgctcagttgccaagaagcatcctaaaacttgggtacattacattgctgctgaagaggaggactgggactatgctcccttagtcctcgcccccgatgacagaagttataaaagtcaatatttgaacaatggccctcagcggattggtaggaagtacaaaaaagtccgatttatggcatacacagatgaaacctttaagactcgtgaagctattcagcatgaatcaggaatcttgggacctttactttatggggaagttggagacacactgttgattatatttaagaatcaagcaagcagaccatataacatctaccctcacggaatcactgatgtccgtcctttgtattcaaggagattaccaaaaggtgtaaaacatttgaaggattttccaattctgccaggagaaatattcaaatataaatggacagtgactgtagaagatgggccaactaaatcagatcctcggtgcctgacccgctattactctagtttcgttaatatggagagagatctagcttcaggactcattggccctctcctcatctgctacaaagaatctgtagatcaaagaggaaaccagataatgtcagacaagaggaatgtcatcctgttttctgtatttgatgagaaccgaagctggtacctcacagagaatatacaacgctttctccccaatccagctggagtgcagcttgaggatccagagttccaagcctccaacatcatgcacagcatcaatggctatgtttttgatagtttgcagttgtcagtttgtttgcatgaggtggcatactggtacattctaagcattggagcacagactgacttcctttctgtcttcttctctggatataccttcaaacacaaaatggtctatgaagacacactcaccctattcccattctcaggagaaactgtcttcatgtcgatggaaaacccaggtctatggattctggggtgccacaactcagactttcggaacagaggcatgaccgccttactgaaggtttctagttgtgacaagaacactggtgattattacgaggacagttatgaagatatttcagcatacttgctgagtaaaaacaatgccattgaaccaagaagcttctcccaaaacccaccagtcttgaaacaccatcaacgggaaataactcgtactactcttcagtcagatcaagaggaaattgactatgatgataccatatcagttgaaatgaagaaggaagattttgacatttatgatgaggatgaaaatcagagcccccgcagctttcaaaagaaaacacgacactattttattgctgcagtggagaggctctgggattatgggatgagtagctccccacatgttctaagaaacagggctcagagtggcagtgtccctcagttcaagaaagttgttttccaggaatttactgatggctcctttactcagcccttataccgtggagaactaaatgaacatttgggactcctggggccatatataagagcagaagttgaagataatatcatggtaactttcagaaatcaggcctctcgtccctattccttctattctagccttatttcttatgaggaagatcagaggcaaggagcagaacctagaaaaaactttgtcaagcctaatgaaaccaaaacttacttttggaaagtgcaacatcatatggcacccactaaagatgagtttgactgcaaagcctgggcttatttctctgatgttgacctggaaaaagatgtgcactcaggcctgattggaccccttctggtctgccacactaacacactgaaccctgctcatgggagacaagtgacagtacaggaatttgctctgtttttcaccatctttgatgagaccaaaagctggtacttcactgaaaatatggaaagaaactgcagggctccctgcaatatccagatggaagatcccacttttaaagagaattatcgcttccatgcaatcaatggctacataatggatacactacctggcttagtaatggctcaggatcaaaggattcgatggtatctgctcagcatgggcagcaatgaaaacatccattctattcatttcagtggacatgtgttcactgtacgaaaaaaagaggagtataaaatggcactgtacaatctctatccaggtgtttttgagacagtggaaatgttaccatccaaagctggaatttggcgggtggaatgccttattggcgagcatctacatgctgggatgagcacactttttctggtgtacagcaataagtgtcagactcccctgggaatggcttctggacacattagagattttcagattacagcttcaggacaatatggacagtgggccccaaagctggccagacttcattattccggatcaatcaatgcctggagcaccaaggagcccttttcttggatcaaggtggatctgttggcaccaatgattattcacggcatcaagacccagggtgcccgtcagaagttctccagcctctacatctctcagtttatcatcatgtatagtcttgatgggaagaagtggcagacttatcgaggaaattccactggaaccttaatggtcttctttggcaatgtggattcatctgggataaaacacaatatttttaaccctccaattattgctcgatacatccgtttgcacccaactcattatagcattcgcagcactcttcgcatggagttgatgggctgtgatttaaatagttgcagcatgccattgggaatggagagtaaagcaatatcagatgcacagattactgcttcatcctactttaccaatatgtttgccacctggtctccttcaaaagctcgacttcacctccaagggaggagtaatgcctggagacctcaggtgaataatccaaaagagtggctgcaagtggacttccagaagacaatgaaagtcacaggagtaactactcagggagtaaaatctctgcttaccagcatgtatgtgaaggagttcctcatctccagcagtcaagatggccatcagtggactctcttttttcagaatggcaaagtaaaggtttttcagggaaatcaagactccttcacacctgtggtgaactctctagacccaccgttactgactcgctaccttcgaattcacccccagagttgggtgcaccagattgccctgaggatggaggttctgggctgcgaggcacaggacctctactga

SEQ ID NO: 10 - DNA, 4374 bp, Artificial Sequence
  source: /note="Description of Artificial Sequence: Synthetic polynucleotide"
atgcaaatagagctctccacctgcttctttctgtgccttttgcgattctgctttagtgccaccagaagatactacctgggtgcagtggaactgtcatgggactatatgcaaagtgatctcggtgagctgcctgtggacgcaagatttcctcctagagtgccaaaatcttttccattcaacacctcagtcgtgtacaaaaagactctgtttgtagaattcacggatcaccttttcaacatcgctaagccaaggccaccctggatgggtctgctaggtcctaccatccaggctgaggtttatgatacagtggtcattacacttaagaacatggcttcccatcctgtcagtcttcatgctgttggtgtatcctactggaaagcttctgagggagctgaatatgatgatcagaccagtcaaagggagaaagaagatgataaagtcttccctggtggaagccatacatatgtctggcaggtcctgaaagagaatggtccaatggcctctgacccactgtgccttacctactcatatctttctcatgtggacctggtaaaagacttgaattcaggcctcattggagccctactagtatgtagagaagggagtctggccaaggaaaagacacagaccttgcacaaatttatactactttttgctgtatttgatgaagggaaaagttggcactcagaaacaaagaactccttgatgcaggatagggatgctgcatctgctcgggcctggcctaaaatgcacacagtcaatggttatgtaaacaggtctctgccaggtctgattggatgccacaggaaatcagtctattggcatgtgattggaatgggcaccactcctgaagtgcactcaatattcctcgaaggtcacacatttcttgtgaggaaccatcgccaggcgtccttggaaatctcgccaataactttccttactgctcaaacactcttgatggaccttggacagtttctactgttttgtcatatctcttcccaccaacatgatggcatggaagcttatgtcaaagtagacagctgtccagaggaaccccaactacgaatgaaaaataatgaagaagcggaagactatgatgatgatcttactgattctgaaatggatgtggtcaggtttgatgatgacaactctccttcctttatccaaattcgctcagttgccaagaagcatcctaaaacttgggtacattacattgctgctgaagaggaggactgggactatgctcccttagtcctcgcccccgatgacagaagttataaaagtcaatatttgaacaatggccctcagcggattggtaggaagtacaaaaaagtccgatttatggcatacacagatgaaacctttaagactcgtgaagctattcagcatgaatcaggaatcttgggacctttactttatggggaagttggagacacactgttgattatatttaagaatcaagcaagcagaccatataacatctaccctcacggaatcactgatgtccgtcctttgtattcaaggagattaccaaaaggtgtaaaacatttgaaggattttccaattctgccaggagaaatattcaaatataaatggacagtgactgtagaagatgggccaactaaatcagatcctcggtgcctgacccgctattactctagtttcgttaatatggagagagatctagcttcaggactcattggccctctcctcatctgctacaaagaatctgtagatcaaagaggaaaccagataatgtcagacaagaggaatgtcatcctgttttctgtatttgatgagaaccgaagctggtacctcacagagaatatacaacgctttctccccaatccagctggagtgcagcttgaggatccagagttccaagcctccaacatcatgcacagcatcaatggctatgtttttgatagtttgcagttgtcagtttgtttgcatgaggtggcatactggtacattctaagcattggagcacagactgacttcctttctgtcttcttctctggatataccttcaaacacaaaatggtctatgaagacacactcaccctattcccattctcaggagaaactgtcttcatgtcgatggaaaacccaggtctatggattctggggtgccacaactcagactttcggaacagaggcatgaccgccttactgaaggtttctagttgtgacaagaacactggtgattattacgaggacagttatgaagatatttcagcatacttgctgagtaaaaacaatgccattgaaccaagaagcttctcccaaaacccaccagtcttgaaagcccatcaagcggaaataactcgtactactcttcagtcagatcaagaggaaattgactatgatgataccatatcagttgaaatgaagaaggaagattttgacatttatgatgaggatgaaaatcagagcccccgcagctttcaaaagaaaacacgacactattttattgctgcagtggagaggctctgggattatgggatgagtagctccccacatgttctaagaaacagggctcagagtggcagtgtccctcagttcaagaaagttgttttccaggaatttactgatggctcctttactcagcccttataccgtggagaactaaatgaacatttgggactcctggggccatatataagagcagaagttgaagataatatcatggtaactttcagaaatcaggcctctcgtccctattccttctattctagccttatttcttatgaggaagatcagaggcaaggagcagaacctagaaaaaactttgtcaagcctaatgaaaccaaaacttacttttggaaagtgcaacatcatatggcacccactaaagatgagtttgactgcaaagcctgggcttatttctctgatgttgacctggaaaaagatgtgcactcaggcctgattggaccccttctggtctgccacactaacacactgaaccctgctcatgggagacaagtgacagtacaggaatttgctctgtttttcaccatctttgatgagaccaaaagctggtacttcactgaaaatatggaaagaaactgcagggctccctgcaatatccagatggaagatcccacttttaaagagaattatcgcttccatgcaatcaatggctacataatggatacactacctggcttagtaatggctcaggatcaaaggattcgatggtatctgctcagcatgggcagcaatgaaaacatccattctattcatttcagtggacatgtgttcactgtacgaaaaaaagaggagtataaaatggcactgtacaatctctatccaggtgtttttgagacagtggaaatgttaccatccaaagctggaatttggcgggtggaatgccttattggcgagcatctacatgctgggatgagcacactttttctggtgtacagcaataagtgtcagactcccctgggaatggcttctggacacattagagattttcagattacagcttcaggacaatatggacagtgggccccaaagctggccagacttcattattccggatcaatcaatgcctggagcaccaaggagcccttttcttggatcaaggtggatctgttggcaccaatgattattcacggcatcaagacccagggtgcccgtcagaagttctccagcctctacatctctcagtttatcatcatgtatagtcttgatgggaagaagtggcagacttatcgaggaaattccactggaaccttaatggtcttctttggcaatgtggattcatctgggataaaacacaatatttttaaccctccaattattgctcgatacatccgtttgcacccaactcattatagcattcgcagcactcttcgcatggagttgatgggctgtgatttaaatagttgcagcatgccattgggaatggagagtaaagcaatatcagatgcacagattactgcttcatcctactttaccaatatgtttgccacctggtctccttcaaaagctcgacttcacctccaagggaggagtaatgcctggagacctcaggtgaataatccaaaagagtggctgcaagtggacttccagaagacaatgaaagtcacaggagtaactactcagggagtaaaatctctgcttaccagcatgtatgtgaaggagttcctcatctccagcagtcaagatggccatcagtggactctcttttttcagaatggcaaagtaaaggtttttcagggaaatcaagactccttcacacctgtggtgaactctctagacccaccgttactgactcgctaccttcgaattcacccccagagttgggtgcaccagattgccctgaggatggaggttctgggctgcgaggcacaggacctctactga

SEQ ID NO: 11 - DNA, 4362 bp, Artificial Sequence
  source: /note="Description of Artificial Sequence: Synthetic polynucleotide"
atgcaaatagagctctccacctgcttctttctgtgccttttgcgattctgctttagtgccaccagaagatactacctgggtgcagtggaactgtcatgggactatatgcaaagtgatctcggtgagctgcctgtggacgcaagatttcctcctagagtgccaaaatcttttccattcaacacctcagtcgtgtacaaaaagactctgtttgtagaattcacggatcaccttttcaacatcgctaagccaaggccaccctggatgggtctgctaggtcctaccatccaggctgaggtttatgatacagtggtcattacacttaagaacatggcttcccatcctgtcagtcttcatgctgttggtgtatcctactggaaagcttctgagggagctgaatatgatgatcagaccagtcaaagggagaaagaagatgataaagtcttccctggtggaagccatacatatgtctggcaggtcctgaaagagaatggtccaatggcctctgacccactgtgccttacctactcatatctttctcatgtggacctggtaaaagacttgaattcaggcctcattggagccctactagtatgtagagaagggagtctggccaaggaaaagacacagaccttgcacaaatttatactactttttgctgtatttgatgaagggaaaagttggcactcagaaacaaagaactccttgatgcaggatagggatgctgcatctgctcgggcctggcctaaaatgcacacagtcaatggttatgtaaacaggtctctgccaggtctgattggatgccacaggaaatcagtctattggcatgtgattggaatgggcaccactcctgaagtgcactcaatattcctcgaaggtcacacatttcttgtgaggaaccatcgccaggcgtccttggaaatctcgccaataactttccttactgctcaaacactcttgatggaccttggacagtttctactgttttgtcatatctcttcccaccaacatgatggcatggaagcttatgtcaaagtagacagctgtccagaggaaccccaactacgaatgaaaaataatgaagaagcggaagactatgatgatgatcttactgattctgaaatggatgtggtcaggtttgatgatgacaactctccttcctttatccaaattcgctcagttgccaagaagcatcctaaaacttgggtacattacattgctgctgaagaggaggactgggactatgctcccttagtcctcgcccccgatgacagaagttataaaagtcaatatttgaacaatggccctcagcggattggtaggaagtacaaaaaagtccgatttatggcatacacagatgaaacctttaagactcgtgaagctattcagcatgaatcaggaatcttgggacctttactttatggggaagttggagacacactgttgattatatttaagaatcaagcaagcagaccatataacatctaccctcacggaatcactgatgtccgtcctttgtattcaaggagattaccaaaaggtgtaaaacatttgaaggattttccaattctgccaggagaaatattcaaatataaatggacagtgactgtagaagatgggccaactaaatcagatcctcggtgcctgacccgctattactctagtttcgttaatatggagagagatctagcttcaggactcattggccctctcctcatctgctacaaagaatctgtagatcaaagaggaaaccagataatgtcagacaagaggaatgtcatcctgttttctgtatttgatgagaaccgaagctggtacctcacagagaatatacaacgctttctccccaatccagctggagtgcagcttgaggatccagagttccaagcctccaacatcatgcacagcatcaatggctatgtttttgatagtttgcagttgtcagtttgtttgcatgaggtggcatactggtacattctaagcattggagcacagactgacttcctttctgtcttcttctctggatataccttcaaacacaaaatggtctatgaagacacactcaccctattcccattctcaggagaaactgtcttcatgtcgatggaaaacccaggtctatggattctggggtgccacaactcagactttcggaacagaggcatgaccgccttactgaaggtttctagttgtgacaagaacactggtgattattacgaggacagttatgaagatatttcagcatacttgctgagtaaaaacaatgccattgaaccaagaagcttctcccaaaacccaccagtcttgaaagaaataactcgtactactcttcagtcagatcaagaggaaattgactatgatgataccatatcagttgaaatgaagaaggaagattttgacatttatgatgaggatgaaaatcagagcccccgcagctttcaaaagaaaacacgacactattttattgctgcagtggagaggctctgggattatgggatgagtagctccccacatgttctaagaaacagggctcagagtggcagtgtccctcagttcaagaaagttgttttccaggaatttactgatggctcctttactcagcccttataccgtggagaactaaatgaacatttgggactcctggggccatatataagagcagaagttgaagataatatcatggtaactttcagaaatcaggcctctcgtccctattccttctattctagccttatttcttatgaggaagatcagaggcaaggagcagaacctagaaaaaactttgtcaagcctaatgaaaccaaaacttacttttggaaagtgcaacatcatatggcacccactaaagatgagtttgactgcaaagcctgggcttatttctctgatgttgacctggaaaaagatgtgcactcaggcctgattggaccccttctggtctgccacactaacacactgaaccctgctcatgggagacaagtgacagtacaggaatttgctctgtttttcaccatctttgatgagaccaaaagctggtacttcactgaaaatatggaaagaaactgcagggctccctgcaatatccagatggaagatcccacttttaaagagaattatcgcttccatgcaatcaatggctacataatggatacactacctggcttagtaatggctcaggatcaaaggattcgatggtatctgctcagcatgggcagcaatgaaaacatccattctattcatttcagtggacatgtgttcactgtacgaaaaaaagaggagtataaaatggcactgtacaatctctatccaggtgtttttgagacagtggaaatgttaccatccaaagctggaatttggcgggtggaatgccttattggcgagcatctacatgctgggatgagcacactttttctggtgtacagcaataagtgtcagactcccctgggaatggcttctggacacattagagattttcagattacagcttcaggacaatatggacagtgggccccaaagctggccagacttcattattccggatcaatcaatgcctggagcaccaaggagcccttttcttggatcaaggtggatctgttggcaccaatgattattcacggcatcaagacccagggtgcccgtcagaagttctccagcctctacatctctcagtttatcatcatgtatagtcttgatgggaagaagtggcagacttatcgaggaaattccactggaaccttaatggtcttctttggcaatgtggattcatctgggataaaacacaatatttttaaccctccaattattgctcgatacatccgtttgcacccaactcattatagcattcgcagcactcttcgcatggagttgatgggctgtgatttaaatagttgcagcatgccattgggaatggagagtaaagcaatatcagatgcacagattactgcttcatcctactttaccaatatgtttgccacctggtctccttcaaaagctcgacttcacctccaagggaggagtaatgcctggagacctcaggtgaataatccaaaagagtggctgcaagtggacttccagaagacaatgaaagtcacaggagtaactactcagggagtaaaatctctgcttaccagcatgtatgtgaaggagttcctcatctccagcagtcaagatggccatcagtggactctcttttttcagaatggcaaagtaaaggtttttcagggaaatcaagactccttcacacctgtggtgaactctctagacccaccgttactgactcgctaccttcgaattcacccccagagttgggtgcaccagattgccctgaggatggaggttctgggctgcgaggcacaggacctctactga

SEQ ID NO: 12 - DNA, 4365 bp, Artificial Sequence
  source: /note="Description of Artificial Sequence: Synthetic polynucleotide"
atgcaaatagagctctccacctgcttctttctgtgccttttgcgattctgctttagtgccaccagaagatactacctgggtgcagtggaactgtcatgggactatatgcaaagtgatctcggtgagctgcctgtggacgcaagatttcctcctagagtgccaaaatcttttccattcaacacctcagtcgtgtacaaaaagactctgtttgtagaattcacggatcaccttttcaacatcgctaagccaaggccaccctggatgggtctgctaggtcctaccatccaggctgaggtttatgatacagtggtcattacacttaagaacatggcttcccatcctgtcagtcttcatgctgttggtgtatcctactggaaagcttctgagggagctgaatatgatgatcagaccagtcaaagggagaaagaagatgataaagtcttccctggtggaagccatacatatgtctggcaggtcctgaaagagaatggtccaatggcctctgacccactgtgccttacctactcatatctttctcatgtggacctggtaaaagacttgaattcaggcctcattggagccctactagtatgtagagaagggagtctggccaaggaaaagacacagaccttgcacaaatttatactactttttgctgtatttgatgaagggaaaagttggcactcagaaacaaagaactccttgatgcaggatagggatgctgcatctgctcgggcctggcctaaaatgcacacagtcaatggttatgtaaacaggtctctgccaggtctgattggatgccacaggaaatcagtctattggcatgtgattggaatgggcaccactcctgaagtgcactcaatattcctcgaaggtcacacatttcttgtgaggaaccatcgccaggcgtccttggaaatctcgccaataactttccttactgctcaaacactcttgatggaccttggacagtttctactgttttgtcatatctcttcccaccaacatgatggcatggaagcttatgtcaaagtagacagctgtccagaggaaccccaactacgaatgaaaaataatgaagaagcggaagactatgatgatgatcttactgattctgaaatggatgtggtcaggtttgatgatgacaactctccttcctttatccaaattcgctcagttgccaagaagcatcctaaaacttgggtacattacattgctgctgaagaggaggactgggactatgctcccttagtcctcgcccccgatgacagaagttataaaagtcaatatttgaacaatggccctcagcggattggtaggaagtacaaaaaagtccgatttatggcatacacagatgaaacctttaagactcgtgaagctattcagcatgaatcaggaatcttgggacctttactttatggggaagttggagacacactgttgattatatttaagaatcaagcaagcagaccatataacatctaccctcacggaatcactgatgtccgtcctttgtattcaaggagattaccaaaaggtgtaaaacatttgaaggattttccaattctgccaggagaaatattcaaatataaatggacagtgactgtagaagatgggccaactaaatcagatcctcggtgcctgacccgctattactctagtttcgttaatatggagagagatctagcttcaggactcattggccctctcctcatctgctacaaagaatctgtagatcaaagaggaaaccagataatgtcagacaagaggaatgtcatcctgttttctgtatttgatgagaaccgaagctggtacctcacagagaatatacaacgctttctccccaatccagctggagtgcagcttgaggatccagagttccaagcctccaacatcatgcacagcatcaatggctatgtttttgatagtttgcagttgtcagtttgtttgcatgaggtggcatactggtacattctaagcattggagcacagactgacttcctttctgtcttcttctctggatataccttcaaacacaaaatggtctatgaagacacactcaccctattcccattctcaggagaaactgtcttcatgtcgatggaaaacccaggtctatggattctggggtgccacaactcagactttcggaacagaggcatgaccgccttactgaaggtttctagttgtgacaagaacactggtgattattacgaggacagttatgaagatatttcagcatacttgctgagtaaaaacaatgccattgaaccaagaagcttctcccaaaacccaccagtcttgaaacgcgaaataactcgtactactcttcagtcagatcaagaggaaattgactatgatgataccatatcagttgaaatgaagaaggaagattttgacatttatgatgaggatgaaaatcagagcccccgcagctttcaaaagaaaacacgacactattttattgctgcagtggagaggctctgggattatgggatgagtagctccccacatgttctaagaaacagggctcagagtggcagtgtccctcagttcaagaaagttgttttccaggaatttactgatggctcctttactcagcccttataccgtggagaactaaatgaacatttgggactcctggggccatatataagagcagaagttgaagataatatcatggtaactttcagaaatcaggcctctcgtccctattccttctattctagccttatttcttatgaggaagatcagaggcaaggagcagaacctagaaaaaactttgtcaagcctaatgaaaccaaaacttacttttggaaagtgcaacatcatatggcacccactaaagatgagtttgactgcaaagcctgggcttatttctctgatgttgacctggaaaaagatgtgcactcaggcctgattggaccccttctggtctgccacactaacacactgaaccctgctcatgggagacaagtgacagtacaggaatttgctctgtttttcaccatctttgatgagaccaaaagctggtacttcactgaaaatatggaaagaaactgcagggctccctgcaatatccagatggaagatcccacttttaaagagaattatcgcttccatgcaatcaatggctacataatggatacactacctggcttagtaatggctcaggatcaaaggattcgatggtatctgctcagcatgggcagcaatgaaaacatccattctattcatttcagtggacatgtgttcactgtacgaaaaaaagaggagtataaaatggcactgtacaatctctatccaggtgtttttgagacagtggaaatgttaccatccaaagctggaatttggcgggtggaatgccttattggcgagcatctacatgctgggatgagcacactttttctggtgtacagcaataagtgtcagactcccctgggaatggcttctggacacattagagattttcagattacagcttcaggacaatatggacagtgggccccaaagctggccagacttcattattccggatcaatcaatgcctggagcaccaaggagcccttttcttggatcaaggtggatctgttggcaccaatgattattcacggcatcaagacccagggtgcccgtcagaagttctccagcctctacatctctcagtttatcatcatgtatagtcttgatgggaagaagtggcagacttatcgaggaaattccactggaaccttaatggtcttctttggcaatgtggattcatctgggataaaacacaatatttttaaccctccaattattgctcgatacatccgtttgcacccaactcattatagcattcgcagcactcttcgcatggagttgatgggctgtgatttaaatagttgcagcatgccattgggaatggagagtaaagcaatatcagatgcacagattactgcttcatcctactttaccaatatgtttgccacctggtctccttcaaaagctcgacttcacctccaagggaggagtaatgcctggagacctcaggtgaataatccaaaagagtggctgcaagtggacttccagaagacaatgaaagtcacaggagtaactactcagggagtaaaatctctgcttaccagcatgtatgtgaaggagttcctcatctccagcagtcaagatggccatcagtggactctcttttttcagaatggcaaagtaaaggtttttcagggaaatcaagactccttcacacctgtggtgaactctctagacccaccgttactgactcgctaccttcgaattcacccccagagttgggtgcaccagattgccctgaggatggaggttctgggctgcgaggcacaggacctctactga

SEQ ID NO: 13 - DNA, 4374 bp, Artificial Sequence
  source: /note="Description of Artificial Sequence: Synthetic polynucleotide"
atgcagatcgagctgtctacctgcttcttcctgtgcctgctgcggttctgcttcagcgccaccagaagatattacctgggcgccgtggaactgagctgggactacatgcagtctgacctgggagagctgcccgtggacgctagatttcctccaagagtgcccaagagcttccccttcaacacctccgtggtgtacaagaaaaccctgttcgtggaattcaccgaccacctgttcaatatcgccaagcctcggcctccttggatgggactgctgggacctacaattcaggccgaggtgtacgacaccgtggtcatcaccctgaagaacatggccagccatcctgtgtctctgcacgccgtgggagtgtcttactggaaggcttctgagggcgccgagtacgacgatcagacaagccagagagagaaagaggacgacaaggttttccctggcggcagccacacctatgtctggcaggtcctgaaagaaaacggccctatggcctccgatcctctgtgcctgacatacagctacctgagccacgtggacctggtcaaggacctgaattctggcctgatcggagccctgctcgtgtgtagagaaggcagcctggccaaagagaaaacccagacactgcacaagttcatcctgctgttcgccgtgttcgacgagggcaagagctggcacagcgagacaaagaacagcctgatgcaggacagggatgccgcctctgctagagcttggcctaagatgcacaccgtgaacggctacgtgaacagaagcctgcctggactgatcggctgccacagaaagtccgtgtactggcacgtgatcggcatgggcacaacacctgaggtgcacagcatctttctggaaggacacaccttcctcgtgcggaaccatagacaggccagcctggaaatcagccctatcaccttcctgaccgctcagaccctgctgatggatctgggccagtttctgctgttctgccacatcagctcccaccagcacgatggcatggaagcctacgtgaaggtggacagctgccccgaagaaccccagctgcggatgaagaacaacgaggaagccgaggactacgacgacgacctgaccgactctgagatggacgtcgtcagattcgacgacgataacagccccagcttcatccagatcagaagcgtggccaagaagcaccccaagacctgggtgcactatatcgccgccgaggaagaggactgggattacgctcctctggtgctggcccctgacgacagaagctacaagagccagtacctgaacaacggccctcagcggatcggccggaagtataagaaagtgcggttcatggcctacaccgacgagacattcaagaccagagaggccatccagcacgagagcggaattctgggccctctgctgtatggcgaagtgggcgatacactgctgatcatcttcaagaaccaggccagcagaccctacaacatctaccctcacggcatcaccgatgtgcggcccctgtattctagaaggctgcccaagggcgtgaagcacctgaaggacttccctatcctgcctggcgagatcttcaagtacaagtggaccgtgaccgtggaagatggccccaccaagagcgaccctagatgtctgacacggtactacagcagcttcgtgaacatggaacgcgacctggccagcggcctgattggacctctgctgatctgctacaaagaaagcgtggaccagcggggcaaccagatcatgagcgacaagcggaacgtgatcctgtttagcgtgttcgatgagaaccggtcctggtatctgaccgagaacatccagcggtttctgcccaatcctgctggcgtgcagctggaagatcctgagttccaggcctccaacatcatgcactccatcaatggctatgtgttcgacagcctgcagctgagcgtgtgcctgcacgaagtggcctactggtacatcctgagcattggcgcccagaccgacttcctgtccgtgttctttagcggctacaccttcaagcacaagatggtgtacgaggataccctgacactgttcccattcagcggcgagacagtgttcatgagcatggaaaaccccggcctgtggatcctgggctgtcacaacagcgacttccggaacagaggcatgacagccctgctgaaggtgtccagctgcgacaagaacaccggcgactactacgaggacagctatgaggacatcagcgcctacctgctgagcaagaacaatgccatcgagcctcggagcttcagccagaatcctcctgtgctgaagcggcaccagcgcgagatcaccagaacaaccctgcagagcgaccaagaggaaatcgattacgacgacaccatcagcgtcgagatgaagaaagaagatttcgacatctacgacgaggacgagaatcagagccccagaagctttcagaaaaagacccggcactacttcattgccgccgtcgagagactgtgggactacggcatgtctagcagccctcacgtgctgagaaatagagcccagagcggcagcgtgccccagttcaagaaagtggtgttccaagagttcaccgacggcagcttcacccagccactgtatagaggcgagctgaacgagcatctgggcctgctgggcccttatatcagagccgaagtggaagataacatcatggtcaccttccggaatcaggcctctcggccctacagcttctacagctccctgatcagctacgaagaggaccagagacagggcgctgagcccagaaagaacttcgtgaagcccaacgagactaagacctacttttggaaggtgcagcaccacatggcccctacaaaggacgagttcgactgcaaggcctgggcctacttttccgatgtggatctggaaaaggacgtgcacagcgggctcatcggaccactgcttgtgtgccacaccaacacactgaaccccgctcacggcagacaagtgacagtgcaagagttcgccctgttcttcaccatcttcgacgaaacaaagagctggtacttcaccgagaatatggaacggaactgcagagccccttgcaacatccagatggaagatcccaccttcaaagagaactaccggttccacgccatcaacggctacatcatggacacactgcccggcctggttatggctcaggatcagagaatccggtggtatctgctgtccatgggctccaacgagaatatccacagcatccacttcagcggccacgtgttcaccgtgcggaaaaaagaagagtacaaaatggccctgtacaatctgtaccctggggtgttcgaaaccgtggaaatgctgccttccaaggccggcatttggagagtggaatgtctgattggagagcacctccacgccggaatgagcaccctgtttctggtgtacagcaacaagtgtcagacccctctcggcatggcctctggacacatcagagacttccagatcaccgcctctggccagtacggacagtgggctcctaaactggctcggctgcactacagcggcagcatcaatgcctggtccaccaaagagcccttcagctggatcaaggtggacctgctggctcccatgatcatccacggaatcaagacccagggcgccagacagaagttcagcagcctgtacatcagccagttcatcatcatgtacagcctggacggcaagaagtggcagacctacagaggcaacagcaccggcacactcatggtgttcttcggcaacgtggactccagcggcattaagcacaacatcttcaaccctccaatcattgcccggtacatccggctgcaccccacacactacagcatccggtctaccctgagaatggaactgatgggctgcgacctgaacagctgcagcatgcccctcggaatggaaagcaaggccatcagcgacgcccagatcacagccagcagctacttcaccaacatgttcgccacttggagcccctccaaggctagactgcatctgcagggcagaagcaacgcttggaggccccaagtgaacaaccccaaagagtggctgcaggtcgactttcaaaagaccatgaaagtgaccggcgtgaccacacagggcgtcaagtctctgctgacctctatgtacgtgaaagagttcctgatctccagcagccaggacggccatcagtggaccctgtttttccagaacggcaaagtgaaagtgttccagggcaatcaggacagcttcacacccgtggtcaactccctggatcctccactgctgaccagatacctgcggattcaccctcagtcttgggtgcaccagatcgctctgcggatggaagtgctgggctgtgaagctcaggacctctactga

SEQ ID NO: 14 - DNA, 4374 bp, Artificial Sequence
  source: /note="Description of Artificial Sequence: Synthetic polynucleotide"
atgcagatcgagctgagcacctgcttcttcctgtgcctgctgcgcttctgcttcagcgccacccgccgctactacctgggcgccgtggagctgagctgggactacatgcagagcgacctgggcgagctgcccgtggacgcccgcttccccccccgcgtgcccaagagcttccccttcaacaccagcgtggtgtacaagaagaccctgttcgtggagttcaccgaccacctgttcaacatcgccaagccccgccccccctggatgggcctgctgggccccaccatccaggccgaggtgtacgacaccgtggtgatcaccctgaagaacatggccagccaccccgtgagcctgcacgccgtgggcgtgagctactggaaggccagcgagggcgccgagtacgacgaccagaccagccagcgcgagaaggaggacgacaaggtgttccccggcggcagccacacctacgtgtggcaggtgctgaaggagaacggccccatggccagcgaccccctgtgcctgacctacagctacctgagccacgtggacctggtgaaggacctgaacagcggcctgatcggcgccctgctggtgtgccgcgagggcagcctggccaaggagaagacccagaccctgcacaagttcatcctgctgttcgccgtgttcgacgagggcaagagctggcacagcgagaccaagaacagcctgatgcaggaccgcgacgccgccagcgcccgcgcctggcccaagatgcacaccgtgaacggctacgtgaaccgcagcctgcccggcctgatcggctgccaccgcaagagcgtgtactggcacgtgatcggcatgggcaccacccccgaggtgcacagcatcttcctggagggccacaccttcctggtgcgcaaccaccgccaggccagcctggagatcagccccatcaccttcctgaccgcccagaccctgctgatggacctgggccagttcctgctgttctgccacatcagcagccaccagcacgacggcatggaggcctacgtgaaggtggacagctgccccgaggagccccagctgcgcatgaagaacaacgaggaggccgaggactacgacgacgacctgaccgacagcgagatggacgtggtgcgcttcgacgacgacaacagccccagcttcatccagatccgcagcgtggccaagaagcaccccaagacctgggtgcactacatcgccgccgaggaggaggactgggactacgcccccctggtgctggcccccgacgaccgcagctacaagagccagtacctgaacaacggcccccagcgcatcggccgcaagtacaagaaggtgcgcttcatggcctacaccgacgagaccttcaagacccgcgaggccatccagcacgagagcggcatcctgggccccctgctgtacggcgaggtgggcgacaccctgctgatcatcttcaagaaccaggccagccgcccctacaacatctacccccacggcatcaccgacgtgcgccccctgtacagccgccgcctgcccaagggcgtgaagcacctgaaggacttccccatcctgcccggcgagatcttcaagtacaagtggaccgtgaccgtggaggacggccccaccaagagcgacccccgctgcctgacccgctactacagcagcttcgtgaacatggagcgcgacctggccagcggcctgatcggccccctgctgatctgctacaaggagagcgtggaccagcgcggcaaccagatcatgagcgacaagcgcaacgtgatcctgttcagcgtgttcgacgagaaccgcagctggtacctgaccgagaacatccagcgcttcctgcccaaccccgccggcgtgcagctggaggaccccgagttccaggccagcaacatcatgcacagcatcaacggctacgtgttcgacagcctgcagctgagcgtgtgcctgcacgaggtggcctactggtacatcctgagcatcggcgcccagaccgacttcctgagcgtgttcttcagcggctacaccttcaagcacaagatggtgtacgaggacaccctgaccctgttccccttcagcggcgagaccgtgttcatgagcatggagaaccccggcctgtggatcctgggctgccacaacagcgacttccgcaaccgcggcatgaccgccctgctgaaggtgagcagctgcgacaagaacaccggcgactactacgaggacagctacgaggacatcagcgcctacctgctgagcaagaacaacgccatcgagccccgcagcttcagccagaacccccccgtgctgaagcgccaccagcgcgagatcacccgcaccaccctgcagagcgaccaggaggagatcgactacgacgacaccatcagcgtggagatgaagaaggaggacttcgacatctacgacgaggacgagaaccagagcccccgcagcttccagaagaagacccgccactacttcatcgccgccgtggagcgcctgtgggactacggcatgagcagcagcccccacgtgctgcgcaaccgcgcccagagcggcagcgtgccccagttcaagaaggtggtgttccaggagttcaccgacggcagcttcacccagcccctgtaccgcggcgagctgaacgagcacctgggcctgctgggcccctacatccgcgccgaggtggaggacaacatcatggtgaccttccgcaaccaggccagccgcccctacagcttctacagcagcctgatcagctacgaggaggaccagcgccagggcgccgagccccgcaagaacttcgtgaagcccaacgagaccaagacctacttctggaaggtgcagcaccacatggcccccaccaaggacgagttcgactgcaaggcctgggcctacttcagcgacgtggacctggagaaggacgtgcacagcggcctgatcggccccctgctggtgtgccacaccaacaccctgaaccccgcccacggccgccaggtgaccgtgcaggagttcgccctgttcttcaccatcttcgacgagaccaagagctggtacttcaccgagaacatggagcgcaactgccgcgccccctgcaacatccagatggaggaccccaccttcaaggagaactaccgcttccacgccatcaacggctacatcatggacaccctgcccggcctggtgatggcccaggaccagcgcatccgctggtacctgctgagcatgggcagcaacgagaacatccacagcatccacttcagcggccacgtgttcaccgtgcgcaagaaggaggagtacaagatggccctgtacaacctgtaccccggcgtgttcgagaccgtggagatgctgcccagcaaggccggcatctggcgcgtggagtgcctgatcggcgagcacctgcacgccggcatgagcaccctgttcctggtgtacagcaacaagtgccagacccccctgggcatggccagcggccacatccgcgacttccagatcaccgccagcggccagtacggccagtgggcccccaagctggcccgcctgcactacagcggcagcatcaacgcctggagcaccaaggagcccttcagctggatcaaggtggacctgctggcccccatgatcatccacggcatcaagacccagggcgcccgccagaagttcagcagcctgtacatcagccagttcatcatcatgtacagcctggacggcaagaagtggcagacctaccgcggcaacagcaccggcaccctgatggtgttcttcggcaacgtggacagcagcggcatcaagcacaacatcttcaacccccccatcatcgcccgctacatccgcctgcaccccacccactacagcatccgcagcaccctgcgcatggagctgatgggctgcgacctgaacagctgcagcatgcccctgggcatggagagcaaggccatcagcgacgcccagatcaccgccagcagctacttcaccaacatgttcgccacctggagccccagcaaggcccgcctgcacctgcagggccgcagcaacgcctggcgcccccaggtgaacaaccccaaggagtggctgcaggtggacttccagaagaccatgaaggtgaccggcgtgaccacccagggcgtgaagagcctgctgaccagcatgtacgtgaaggagttcctgatcagcagcagccaggacggccaccagtggaccctgttcttccagaacggcaaggtgaaggtgttccagggcaaccaggacagcttcacccccgtggtgaacagcctggacccccccctgctgacccgctacctgcgcatccacccccagagctgggtgcaccagatcgccctgcgcatggaggtgctgggctgcgaggcccaggacctgtactga

SEQ ID NO: 15 - DNA, 4374 bp, Artificial Sequence
  source: /note="Description of Artificial Sequence: Synthetic polynucleotide"
atgcagattgagctgagcacctgtttcttcctgtgcctgctgagattttgcttctcagctacccgcaggtactacctgggagccgttgagctgtcctgggattacatgcagtcagatctgggggagctgcctgtggacgctcggtttccccccagagtgccaaagtcctttcccttcaacaccagcgtggtgtacaaaaagacactttttgttgaatttactgaccacttgttcaacatcgccaagccacgacccccatggatgggcctgctggggccaaccattcaggcagaggtttacgacacagtcgtgatcacactgaagaacatggcctcccatccagtgtctctgcacgccgtcggtgtgtcctactggaaagcatccgagggcgccgagtatgacgaccagaccagccagagagagaaagaggacgacaaagtgttccctggaggcagccacacctacgtgtggcaggtgttgaaggaaaatgggcccatggccagtgaccctttgtgtctgacttactcatacctgtctcatgtggatctagtcaaggacctgaattctggactgattggggcactgcttgtgtgccgcgaaggcagcctggccaaagaaaagacacagacccttcacaagttcatcctgctgttcgccgtgttcgacgaaggcaaatcctggcactcagaaaccaaaaactcactgatgcaggaccgggatgccgcctctgcccgcgcatggccaaaaatgcacaccgtcaacggctatgtcaatagaagtttgcccggcctcattggatgtcacaggaaaagcgtctattggcatgtaatcgggatgggaaccacacctgaggtccacagcatatttctggaaggccacacatttctggtgagaaatcatcgccaggcttccctggaaatttcccccatcaccttcttgaccgcccagacactgctcatggatcttgggcagtttctgctgttttgtcatatttcttctcaccaacacgacggaatggaggcctacgttaaggtcgatagttgccctgaagaacctcagctgaggatgaagaacaacgaggaagccgaggactacgatgacgatttgaccgattccgaaatggacgtggtgcgctttgatgatgacaattctccatccttcattcagattagatccgtcgccaagaagcaccccaagacctgggtgcactacattgcagccgaggaggaggattgggactacgcccccctggtgctggcacccgacgaccgaagctacaaatctcagtacctgaacaatggtccacaacggatcggcaggaagtacaagaaagtgcggttcatggcctatacagacgaaaccttcaaaaccagggaggctatccagcacgagtctgggattctgggaccactcctgtacggcgaagtgggcgacaccttgttaattatcttcaagaaccaggctagtagaccttataacatttatccccacggcattaccgatgtgcggcctctctactctaggcggcttccaaagggggtgaaacacctgaaggactttcccatcctccctggcgaaatctttaagtataagtggacagtgaccgtggaggatggaccaaccaagagcgaccccaggtgcctgacacgctattattcaagcttcgtgaatatggaaagggacctcgcatctggcttgatcggccctctgctgatatgttacaaggaaagcgtcgatcagagaggaaatcagatcatgtcagacaaaaggaatgtgatcctgttctccgtcttcgatgaaaacaggagctggtatctgacagagaacatccagagattcctgccaaatcccgccggcgtccagctggaggacccggagtttcaggcatctaacatcatgcattccattaatggttacgtgttcgactccctgcagctgagcgtgtgcctccacgaggtggcctactggtacatcttgagcatcggcgcccagaccgactttctgagcgtctttttctccgggtatactttcaaacataagatggtgtacgaagatactctgacgctgttccctttctctggggagactgtgtttatgtctatggagaaccctggactgtggattctcggatgccacaacagtgactttcgtaatagagggatgactgcactgctgaaggtgtccagctgtgataaaaatactggcgactactacgaagatagctatgaggatatctcagcatacctgctgagcaagaataacgccatcgagccccgaagcttctcacagaatccccctgtcctcaagaggcaccagcgagagatcacaaggaccacactccagtccgaccaggaggagattgactacgatgacacgatttctgtggagatgaaaaaagaggactttgacatctacgatgaggatgaaaaccagagccctaggtcgttccagaagaaaacaaggcactacttcattgccgccgtggagagactgtgggactacggaatgagtagttccccacacgtgttgcggaacagagcccagagtgggtccgtcccacagttcaagaaggttgttttccaggagttcacagatggctccttcactcagccactgtatcgcggcgagctgaatgagcacttgggcttattgggcccctacattcgcgcagaagtcgaagataatattatggtgaccttccgcaaccaggccagccggccttactcattctactcctctctcatctcttatgaggaggatcagcgccagggcgccgaaccccggaagaactttgtgaagcccaatgaaaccaaaacttacttttggaaggtgcagcaccatatggcgccgacgaaagacgaatttgactgcaaagcctgggcctacttcagcgacgtcgacttggagaaggacgtccacagcggcctgattggccctttgttggtctgccataccaatacactcaaccctgcccacgggaggcaggtgaccgtgcaggagtttgccttgttcttcaccatcttcgacgaaaccaagagctggtacttcacagagaacatggagaggaactgcagagcaccctgtaacatccagatggaggaccctactttcaaggaaaattacaggttccatgccattaatggctacatcatggataccctccccgggcttgtgatggctcaggaccagcgcatccgctggtacctgctctcaatgggctccaacgagaacattcatagcatccactttagtggccacgtgtttaccgtgcgcaagaaggaggagtacaagatggcactgtacaacctgtaccctggcgtgtttgagacagtggagatgctgccatccaaggccggcatctggcgcgtggagtgcctcattggggagcacctccatgctggcatgtctacactgttcctggtgtacagcaacaagtgtcagactccactcggaatggcctccgggcatatccgcgattttcagatcacggcctctggccagtatggccaatgggctcccaagctggccaggctgcactacagtgggagtatcaacgcttggagcaccaaggagcctttctcctggatcaaggtggacctgcttgcccccatgattattcacggcattaagacacagggggccaggcagaaattctcctccctgtacatctcccagttcatcatcatgtacagtctggacggcaaaaagtggcagacctaccgcgggaacagtaccgggacattgatggtgttcttcgggaacgtggactctagcggcattaaacacaacattttcaacccccccatcattgctaggtatatcaggctccatcccacccactatagcatcaggtccactctgcggatggagctgatgggctgcgaccttaattcatgcagcatgccgctgggcatggagtcaaaggccatctccgacgcccaaatcaccgcctccagctacttcaccaatatgttcgccacctggagccccagcaaggcccggctgcacctgcagggccgcagcaacgcctggcggcctcaggtgaacaaccccaaggagtggctgcaggtggacttccagaaaaccatgaaggtgactggggtcaccacccagggagtcaagagcctgctgaccagcatgtatgtgaaggagttcttgatcagctcgtcacaggatggccaccagtggactttgttctttcagaacggtaaggtgaaagtgttccagggaaaccaagattcctttacaccagtggtcaactctctggatcctcccctgctgacacggtacctgcggatccatccccagtcatgggtgcaccagattgctctgcgcatggaggtgcttggctgcgaggcccaggacctgtactga

SEQ ID NO: 16 - DNA, 4374 bp, Artificial Sequence
  source: /note="Description of Artificial Sequence: Synthetic polynucleotide"
atgcagattgagctgagcacctgtttcttcctgtgcctgctgagattttgcttctcagctacccgcaggtactacctgggagccgttgagctgtcctgggattacatgcagtcagatctgggggagctgcctgtggacgctcggtttccccccagagtgccaaagtcctttcccttcaacaccagcgtggtgtacaaaaagacactttttgttgaatttactgaccacttgttcaacatcgccaagccacgacccccatggatgggcctgctggggccaaccattcaggcagaggtttacgacacagtcgtgatcacactgaagaacatggcctcccatccagtgtctctgcacgccgtcggtgtgtcctactggaaagcatccgagggcgccgagtatgacgaccagaccagccagagagagaaagaggacgacaaagtgttccctggaggcagccacacctacgtgtggcaggtgttgaaggaaaatgggcccatggccagtgaccctttgtgtctgacttactcatacctgtctcatgtggatctagtcaaggacctgaattctggactgattggggcactgcttgtgtgccgcgaaggcagcctggccaaagaaaagacacagacccttcacaagttcatcctgctgttcgccgtgttcgacgaaggcaaatcctggcactcagaaaccaaaaactcactgatgcaggaccgggatgccgcctctgcccgcgcatggccaaaaatgcacaccgtcaacggctatgtcaatagaagtttgcccggcctcattggatgtcacaggaaaagcgtctattggcatgtaatcgggatgggaaccacacctgaggtccacagcatatttctggaaggccacacatttctggtgagaaatcatcgccaggcttccctggaaatttcccccatcaccttcttgaccgcccagacactgctcatggatcttgggcagtttctgctgttttgtcatatttcttctcaccaacacgacggaatggaggcctacgttaaggtcgatagttgccctgaagaacctcagctgaggatgaagaacaacgaggaagccgaggactacgatgacgatttgaccgattccgaaatggacgtggtgcgctttgatgatgacaattctccatccttcattcagattagatccgtcgccaagaagcaccccaagacctgggtgcactacattgcagccgaggaggaggattgggactacgcccccctggtgctggcacccgacgaccgaagctacaaatctcagtacctgaacaatggtccacaacggatcggcaggaagtacaagaaagtgcggttcatggcctatacagacgaaaccttcaaaaccagggaggctatccagcacgagtctgggattctgggaccactcctgtacggcgaagtgggcgacaccttgttaattatcttcaagaaccaggctagtagaccttataacatttatccccacggcattaccgatgtgcggcctctctactctaggcggcttccaaagggggtgaaacacctgaaggactttcccatcctccctggcgaaatctttaagtataagtggacagtgaccgtggaggatggaccaaccaagagcgaccccaggtgcctgacacgctattattcaagcttcgtgaatatggaaagggacctcgcatctggcttgatcggccctctgctgatatgttacaaggaaagcgtcgatcagagaggaaatcagatcatgtcagacaaaaggaatgtgatcctgttctccgtcttcgatgaaaacaggagctggtatctgacagagaacatccagagattcctgccaaatcccgccggcgtccagctggaggacccggagtttcaggcatctaacatcatgcattccattaatggttacgtgttcgactccctgcagctgagcgtgtgcctccacgaggtggcctactggtacatcttgagcatcggcgcccagaccgactttctgagcgtctttttctccgggtatactttcaaacataagatggtgtacgaagatactctgacgctgttccctttctctggggagactgtgtttatgtctatggagaaccctggactgtggattctcggatgccacaacagtgactttcgtaatagagggatgactgcactgctgaaggtgtccagctgtgataaaaatactggcgactactacgaagatagctatgaggatatctcagcatacctgctgagcaagaataacgccatcgagccccgaagcttctcacagaatccccctgtcctcaaggcccaccaggcggagatcacaaggaccacactccagtccgaccaggaggagattgactacgatgacacgatttctgtggagatgaaaaaagaggactttgacatctacgatgaggatgaaaaccagagccctaggtcgttccagaagaaaacaaggcactacttcattgccgccgtggagagactgtgggactacggaatgagtagttccccacacgtgttgcggaacagagcccagagtgggtccgtcccacagttcaagaaggttgttttccaggagttcacagatggctccttcactcagccactgtatcgcggcgagctgaatgagcacttgggcttattgggcccctacattcgcgcagaagtcgaagataatattatggtgaccttccgcaaccaggccagccggccttactcattctactcctctctcatctcttatgaggaggatcagcgccagggcgccgaaccccggaagaactttgtgaagcccaatgaaaccaaaacttacttttggaaggtgcagcaccatatggcgccgacgaaagacgaatttgactgcaaagcctgggcctacttcagcgacgtcgacttggagaaggacgtccacagcggcctgattggccctttgttggtctgccataccaatacactcaaccctgcccacgggaggcaggtgaccgtgcaggagtttgccttgttcttcaccatcttcgacgaaaccaagagctggtacttcacagagaacatggagaggaactgcagagcaccctgtaacatccagatggaggaccctactttcaaggaaaattacaggttccatgccattaatggctacatcatggataccctccccgggcttgtgatggctcaggaccagcgcatccgctggtacctgctctcaatgggctccaacgagaacattcatagcatccactttagtggccacgtgtttaccgtgcgcaagaaggaggagtacaagatggcactgtacaacctgtaccctggcgtgtttgagacagtggagatgctgccatccaaggccggcatctggcgcgtggagtgcctcattggggagcacctccatgctggcatgtctacactgttcctggtgtacagcaacaagtgtcagactccactcggaatggcctccgggcatatccgcgattttcagatcacggcctctggccagtatggccaatgggctcccaagctggccaggctgcactacagtgggagtatcaacgcttggagcaccaaggagcctttctcctggatcaaggtggacctgcttgcccccatgattattcacggcattaagacacagggggccaggcagaaattctcctccctgtacatctcccagttcatcatcatgtacagtctggacggcaaaaagtggcagacctaccgcgggaacagtaccgggacattgatggtgttcttcgggaacgtggactctagcggcattaaacacaacattttcaacccccccatcattgctaggtatatcaggctccatcccacccactatagcatcaggtccactctgcggatggagctgatgggctgcgaccttaattcatgcagcatgccgctgggcatggagtcaaaggccatctccgacgcccaaatcaccgcctccagctacttcaccaatatgttcgccacctggagccccagcaaggcccggctgcacctgcagggccgcagcaacgcctggcggcctcaggtgaacaaccccaaggagtggctgcaggtggacttccagaaaaccatgaaggtgactggggtcaccacccagggagtcaagagcctgctgaccagcatgtatgtgaaggagttcttgatcagctcgtcacaggatggccaccagtggactttgttctttcagaacggtaaggtgaaagtgttccagggaaaccaagattcctttacaccagtggtcaactctctggatcctcccctgctgacacggtacctgcggatccatccccagtcatgggtgcaccagattgctctgcgcatggaggtgcttggctgcgaggcccaggacctgtactga

SEQ ID NO: 17 - DNA, 4425 bp, Artificial Sequence
  source: /note="Description of Artificial Sequence: Synthetic polynucleotide"
atgcagattgagctgagcacctgtttcttcctgtgcctgctgagattttgcttctcagctacccgcaggtactacctgggagccgttgagctgtcctgggattacatgcagtcagatctgggggagctgcctgtggacgctcggtttccccccagagtgccaaagtcctttcccttcaacaccagcgtggtgtacaaaaagacactttttgttgaatttactgaccacttgttcaacatcgccaagccacgacccccatggatgggcctgctggggccaaccattcaggcagaggtttacgacacagtcgtgatcacactgaagaacatggcctcccatccagtgtctctgcacgccgtcggtgtgtcctactggaaagcatccgagggcgccgagtatgacgaccagaccagccagagagagaaagaggacgacaaagtgttccctggaggcagccacacctacgtgtggcaggtgttgaaggaaaatgggcccatggccagtgaccctttgtgtctgacttactcatacctgtctcatgtggatctagtcaaggacctgaattctggactgattggggcactgcttgtgtgccgcgaaggcagcctggccaaagaaaagacacagacccttcacaagttcatcctgctgttcgccgtgttcgacgaaggcaaatcctggcactcagaaaccaaaaactcactgatgcaggaccgggatgccgcctctgcccgcgcatggccaaaaatgcacaccgtcaacggctatgtcaatagaagtttgcccggcctcattggatgtcacaggaaaagcgtctattggcatgtaatcgggatgggaaccacacctgaggtccacagcatatttctggaaggccacacatttctggtgagaaatcatcgccaggcttccctggaaatttcccccatcaccttcttgaccgcccagacactgctcatggatcttgggcagtttctgctgttttgtcatatttcttctcaccaacacgacggaatggaggcctacgttaaggtcgatagttgccctgaagaacctcagctgaggatgaagaacaacgaggaagccgaggactacgatgacgatttgaccgattccgaaatggacgtggtgcgctttgatgatgacaattctccatccttcattcagattagatccgtcgccaagaagcaccccaagacctgggtgcactacattgcagccgaggaggaggattgggactacgcccccctggtgctggcacccgacgaccgaagctacaaatctcagtacctgaacaatggtccacaacggatcggcaggaagtacaagaaagtgcggttcatggcctatacagacgaaaccttcaaaaccagggaggctatccagcacgagtctgggattctgggaccactcctgtacggcgaagtgggcgacaccttgttaattatcttcaagaaccaggctagtagaccttataacatttatccccacggcattaccgatgtgcggcctctctactctaggcggcttccaaagggggtgaaacacctgaaggactttcccatcctccctggcgaaatctttaagtataagtggacagtgaccgtggaggatggaccaaccaagagcgaccccaggtgcctgacacgctattattcaagcttcgtgaatatggaaagggacctcgcatctggcttgatcggccctctgctgatatgttacaaggaaagcgtcgatcagagaggaaatcagatcatgtcagacaaaaggaatgtgatcctgttctccgtcttcgatgaaaacaggagctggtatctgacagagaacatccagagattcctgccaaatcccgccggcgtccagctggaggacccggagtttcaggcatctaacatcatgcattccattaatggttacgtgttcgactccctgcagctgagcgtgtgcctccacgaggtggcctactggtacatcttgagcatcggcgcccagaccgactttctgagcgtctttttctccgggtatactttcaaacataagatggtgtacgaagatactctgacgctgttccctttctctggggagactgtgtttatgtctatggagaaccctggactgtggattctcggatgccacaacagtgactttcgtaatagagggatgactgcactgctgaaggtgtccagctgtgataaaaatactggcgactactacgaagatagctatgaggatatctcagcatacctgctgagcaagaataacgccatcgagccccgaagcttctcacagaatgccaccaacgtgagcaacaacagcaacaccagcaacgacagcaacgtgagcccccctgtcctcaaggcccaccaggcggagatcacaaggaccacactccagtccgaccaggaggagattgactacgatgacacgatttctgtggagatgaaaaaagaggactttgacatctacgatgaggatgaaaaccagagccctaggtcgttccagaagaaaacaaggcactacttcattgccgccgtggagagactgtgggactacggaatgagtagttccccacacgtgttgcggaacagagcccagagtgggtccgtcccacagttcaagaaggttgttttccaggagttcacagatggctccttcactcagccactgtatcgcggcgagctgaatgagcacttgggcttattgggcccctacattcgcgcagaagtcgaagataatattatggtgaccttccgcaaccaggccagccggccttactcattctactcctctctcatctcttatgaggaggatcagcgccagggcgccgaaccccggaagaactttgtgaagcccaatgaaaccaaaacttacttttggaaggtgcagcaccatatggcgccgacgaaagacgaatttgactgcaaagcctgggcctacttcagcgacgtcgacttggagaaggacgtccacagcggcctgattggccctttgttggtctgccataccaatacactcaaccctgcccacgggaggcaggtgaccgtgcaggagtttgccttgttcttcaccatcttcgacgaaaccaagagctggtacttcacagagaacatggagaggaactgcagagcaccctgtaacatccagatggaggaccctactttcaaggaaaattacaggttccatgccattaatggctacatcatggataccctccccgggcttgtgatggctcaggaccagcgcatccgctggtacctgctctcaatgggctccaacgagaacattcatagcatccactttagtggccacgtgtttaccgtgcgcaagaaggaggagtacaagatggcactgtacaacctgtaccctggcgtgtttgagacagtggagatgctgccatccaaggccggcatctggcgcgtggagtgcctcattggggagcacctccatgctggcatgtctacactgttcctggtgtacagcaacaagtgtcagactccactcggaatggcctccgggcatatccgcgattttcagatcacggcctctggccagtatggccaatgggctcccaagctggccaggctgcactacagtgggagtatcaacgcttggagcaccaaggagcctttctcctggatcaaggtggacctgcttgcccccatgattattcacggcattaagacacagggggccaggcagaaattctcctccctgtacatctcccagttcatcatcatgtacagtctggacggcaaaaagtggcagacctaccgcgggaacagtaccgggacattgatggtgttcttcgggaacgtggactctagcggcattaaacacaacattttcaacccccccatcattgctaggtatatcaggctccatcccacccactatagcatcaggtccactctgcggatggagctgatgggctgcgaccttaattcatgcagcatgccgctgggcatggagtcaaaggccatctccgacgcccaaatcaccgcctccagctacttcaccaatatgttcgccacctggagccccagcaaggcccggctgcacctgcagggccgcagcaacgcctggcggcctcaggtgaacaaccccaaggagtggctgcaggtggacttccagaaaaccatgaaggtgactggggtcaccacccagggagtcaagagcctgctgaccagcatgtatgtgaaggagttcttgatcagctcgtcacaggatggccaccagtggactttgttctttcagaacggtaaggtgaaagtgttccagggaaaccaagattcctttacaccagtggtcaactctctggatcctcccctgctgacacggtacctgcggatccatccccagtcatgggtgcaccagattgctctgcgcatggaggtgcttggctgcgaggcccaggacctgtactaa

SEQ ID NO: 18 - DNA, 1386 bp, Artificial Sequence
  source: /note="Description of Artificial Sequence: Synthetic polynucleotide"
atgcagcgcgtgaacatgatcatggcagaatcaccaggcctcatcaccatctgccttttaggatatctactcagtgctgaatgtacagtttttcttgatcatgaaaacgccaacaaaattctgaatcggccaaagaggtataattcaggtaaattggaagagtttgttcaagggaaccttgagagagaatgtatggaagaaaagtgtagttttgaagaagcacgagaagtttttgaaaacactgaaagaacaactgaattttggaagcagtatgttgatggagatcagtgtgagtccaatccatgtttaaatggcggcagttgcaaggatgacattaattcctatgaatgttggtgtccctttggatttgaaggaaagaactgtgaattagatgtaacatgtaacattaagaatggcagatgcgagcagttttgtaaaaatagtgctgataacaaggtggtttgctcctgtactgagggatatcgacttgcagaaaaccagaagtcctgtgaaccagcagtgccatttccatgtggaagagtttctgtttcacaaacttctaagctcacccgtgctgagactgtttttcctgatgtggactatgtaaattctactgaagctgaaaccattttggataacatcactcaaagcacccaatcatttaatgacttcactcgggttgttggtggagaagatgccaaaccaggtcaattcccttggcaggttgttttgaatggtaaagttgatgcattctgtggaggctctatcgttaatgaaaaatggattgtaactgctgcccactgtgttgaaactggtgttaaaattacagttgtcgcaggtgaacataatattgaggagacagaacatacagagcaaaagcgaaatgtgattcgaattattcctcaccacaactacaatgcagctattaataagtacaaccatgacattgcccttctggaactggacgaacccttagtgctaaacagctacgttacacctatttgcattgctgacaaggaatacacgaacatcttcctcaaatttggatctggctatgtaagtggctggggaagagtcttccacaaagggagatcagctttagttcttcagtaccttagagttccacttgttgaccgagccacatgtcttctgtctacaaagttcaccatctataacaacatgttctgtgctggcttccatgaaggaggtagagattcatgtcaaggagatagtgggggaccccatgttactgaagtggaagggaccagtttcttaactggaattattagctggggtgaagagtgtgcaatgaaaggcaaatatggaatatataccaaggtatcccggtatgtcaactggattaaggaaaaaacaaagctcacttaa

SEQ ID NO: 19 - DNA, 1386 bp, Artificial Sequence
  source: /note="Description of Artificial Sequence: Synthetic polynucleotide"
atgcagcgcgtgaacatgattatggccgagtctcccggcctgatcaccatctgtctgctgggctatctgctgagcgccgagtgcaccgtgtttctggatcacgagaacgccaacaagatcctgaacagacccaagcggtacaacagcggcaagctggaagagttcgtgcagggcaacctggaacgcgagtgcatggaagagaagtgcagcttcgaagaggccagagaggtgttcgagaacaccgagagaaccaccgagttctggaagcagtacgtggacggcgatcagtgcgagagcaacccttgtctgaatggcggcagctgcaaggacgacatcaacagctacgagtgctggtgccccttcggcttcgagggcaagaattgcgagctggacgtgacctgcaacatcaagaacggcagatgcgagcagttctgcaagaacagcgccgacaacaaggtcgtgtgctcctgcacagagggctacagactggccgagaaccagaagtcttgcgagcccgctgtgccctttccatgtggcagagtgtctgtgtcccagaccagcaagctgaccagagccgagacagtgttccccgacgtggactacgtgaacagcaccgaggccgagacaatcctggacaacatcacccagagcacccagtccttcaacgacttcaccagagtcgtcggcggcgaggatgctaagcctggacagtttccttggcaagtggtgctgaacggcaaggtggacgctttttgtggcggctccatcgtgaacgagaagtggatcgtgaccgccgctcactgtgtggaaaccggcgtgaagattacagtggtggccggcgagcacaacatcgaggaaacagagcacaccgagcagaaacggaacgtgatcagaatcatccctcaccacaactacaacgccgccatcaacaagtacaaccacgatatcgccctgctggaactggacgagcccctggtcctgaactcttacgtgacccctatctgtatcgccgacaaagagtacaccaacatctttctgaagttcggcagcggctacgtgtccggctggggaagagttttccacaagggcagatcagccctggtgctgcagtacctgagagtgcccctggtggatagagccacatgcctgctgagcaccaagttcaccatctacaacaacatgttctgcgccggcttccacgaaggcggcagagattcttgtcaaggcgattctggcggccctcacgtgacagaggttgagggcacaagctttctgaccggcatcatcagctggggcgaagagtgtgccatgaaggggaagtacggcatctacaccaaggtgtccagatacgtgaactggatcaaagaaaagaccaagctcacctga

SEQ ID NO: 20 - DNA, 1386 bp, Artificial Sequence
  source: /note="Description of Artificial Sequence: Synthetic polynucleotide"
atgcagcgcgtgaacatgatcatggccgagagccccggcctgatcaccatctgcctgctgggctacctgctgagcgccgagtgcaccgtgttcctggaccacgagaacgccaacaagatcctgaaccgccccaagcgctacaacagcggcaagctggaggagttcgtgcagggcaacctggagcgcgagtgcatggaggagaagtgcagcttcgaggaggcccgcgaggtgttcgagaacaccgagcgcaccaccgagttctggaagcagtacgtggacggcgaccagtgcgagagcaacccctgcctgaacggcggcagctgcaaggacgacatcaacagctacgagtgctggtgccccttcggcttcgagggcaagaactgcgagctggacgtgacctgcaacatcaagaacggccgctgcgagcagttctgcaagaacagcgccgacaacaaggtggtgtgcagctgcaccgagggctaccgcctggccgagaaccagaagagctgcgagcccgccgtgcccttcccctgcggccgcgtgagcgtgagccagaccagcaagctgacccgcgccgagactgtgttccccgacgtggactacgtgaacagcaccgaggccgaaacgatcctggacaacatcacccagagcacccagagcttcaacgacttcacccgcgtggtgggcggcgaggacgccaagcccggccagttcccctggcaggtggtgctgaacggcaaggtggacgccttctgcggcggcagcatcgtgaacgagaagtggatcgtgaccgccgcccactgcgtggaaaccggcgtgaagatcaccgtggtggccggcgagcacaacatcgaggaaaccgagcacaccgagcagaagcgcaacgtgatccgcatcatcccccaccacaactacaacgccgccatcaacaagtacaaccacgacatcgccctgctggagctggacgagcccctggtgctgaacagctacgtgacccccatctgcatcgccgacaaggagtacaccaacatcttcctgaagttcggcagcggctacgtgagcggctggggccgcgtgttccacaagggccgcagcgccctggtgctgcagtacctgcgcgtgcccctggtggaccgcgccacctgcctgctgagcaccaagttcaccatctacaacaacatgttctgcgccggcttccacgagggcggccgcgacagctgccagggcgacagcggcggcccccacgtgaccgaggtggagggcaccagcttcctgaccggcatcatcagctggggcgaggagtgcgccatgaagggcaagtacggcatctacaccaaggtgagccgctacgtgaactggatcaaggagaaaaccaagctgacctaa

SEQ ID NO: 21 - DNA, 1386 bp, Artificial Sequence
  source: /note="Description of Artificial Sequence: Synthetic polynucleotide"
atgcagcgggtgaacatgatcatggccgagagccccgggctgatcaccatctgtctgctggggtacctgctgtccgccgagtgcaccgtgttcctggaccacgagaacgccaacaagatcctgaatcgccccaagagatacaattccggaaagctggaagagtttgtgcagggcaacctggagagagagtgcatggaagagaagtgctccttcgaggaggcccgggaggtgttcgagaatactgaacggacaacagagttctggaagcagtatgtggacggcgaccagtgtgagagcaacccctgtctgaacggcgggagctgcaaggacgacattaattcctacgaatgctggtgcccattcggcttcgagggcaagaactgcgagctggacgtgacctgcaacatcaagaacggccgctgcgagcagttttgcaagaactccgccgacaacaaggtggtgtgttcttgcaccgagggctaccgcctggccgaaaaccagaagagctgtgagcctgccgtgcccttcccctgcggccgggtgtctgtgtcccagacctccaagctgaccagagccgaaaccgtgtttccagatgtggactacgtgaatagcaccgaggccgagactatcctcgacaacatcacccagtccacccagagctttaacgacttcacccgcgtggtgggcggcgaggacgccaagcccggccagttcccctggcaggtggtgctcaacggaaaggtggacgccttctgcggaggcagcatcgtgaatgaaaagtggatcgtgacagccgcccactgcgtggaaacaggggtgaagatcaccgtggtggctggagagcacaacatcgaggagacagagcacaccgaacagaagaggaatgtgatcaggatcatcccccaccacaactataatgccgccatcaacaagtacaaccacgacatcgccctgctggagctggatgagcccctggtgctcaacagctacgtgacccccatctgcatcgctgacaaggagtacaccaacatcttcctgaagttcggctccggctacgtgtctggctggggccgcgtgttccacaagggaagaagcgccctcgtgctgcagtacctgcgggtgccactggtggacagggccacctgcctgctgagcactaagttcaccatttacaacaacatgttctgcgccggcttccacgagggcggcagggactcctgccagggcgacagcggcggcccccatgtgaccgaggtggagggcacctcctttctgactggcattatctcctggggcgaggagtgcgccatgaaggggaagtatggcatctacaccaaggtgtcccgctacgtgaactggattaaggagaaaaccaagctgacctga

SEQ ID NO: 22 - DNA, 313 bp, Artificial Sequence
  source: /note="Description of Artificial Sequence: Synthetic polynucleotide"
ttaaccctagaaagatagtctgcgtaaaattgacgcatgcattcttgaaatattgctctctctttctaaatagcgcgaatccgtcgctgtgcatttaggacatctcagtcgccgcttggagctcccgtgaggcgtgcttgtcaatgcggtaagtgtcactgattttgaactataacgaccgcgtgagtcaaaatgacgcatgattatcttttacgtgacttttaagatttaactcatacgataattatattgttatttcatgttctacttacgtgataacttattatatatatattttcttgttatagatatc

SEQ ID NO: 23 - DNA, 1733 bp, Artificial Sequence
  source: /note="Description of Artificial Sequence: Synthetic polynucleotide"
ctcgacattgattattgactagttattaatagtaatcaattacggggtcattagttcatagcccatatatggagttccgcgttacataacttacggtaaatggcccgcctggctgaccgcccaacgacccccgcccattgacgtcaataatgacgtatgttcccatagtaacgccaatagggactttccattgacgtcaatgggtggagtatttacggtaaactgcccacttggcagtacatcaagtgtatcatatgccaagtacgccccctattgacgtcaatgacggtaaatggcccgcctggcattatgcccagtacatgaccttatgggactttcctacttggcagtacatctacgtattagtcatcgctattaccatggtcgaggtgagccccacgttctgcttcactctccccatctcccccccctccccacccccaattttgtatttatttattttttaattattttgtgcagcgatgggggcggggggggggggggggcgcgcgccaggcggggcggggcggggcgaggggcggggcggggcgaggcggagaggtgcggcggcagccaatcagagcggcgcgctccgaaagtttccttttatggcgaggcggcggcggcggcggccctataaaaagcgaagcgcgcggcgggcgggagtcgctgcgcgctgccttcgccccgtgccccgctccgccgccgcctcgcgccgcccgccccggctctgactgaccgcgttactcccacaggtgagcgggcgggacggcccttctcctccgggctgtaattagcgcttggtttaatgacggcttgtttcttttctgtggctgcgtgaaagccttgaggggctccgggagggccctttgtgcggggggagcggctcggggggtgcgtgcgtgtgtgtgtgcgtggggagcgccgcgtgcggctccgcgctgcccggcggctgtgagcgctgcgggcgcggcgcggggctttgtgcgctccgcagtgtgcgcgaggggagcgcggccgggggcggtgccccgcggtgcggggggggctgcgaggggaacaaaggctgcgtgcggggtgtgtgcgtgggggggtgagcagggggtgtgggcgcgtcggtcgggctgcaaccccccctgcacccccctccccgagttgctgagcacggcccggcttcgggtgcggggctccgtacggggcgtggcgcggggctcgccgtgccgggcggggggtggcggcaggtgggggtgccgggcggggcggggccgcctcgggccggggagggctcgggggaggggcgcggcggcccccggagcgccggcggctgtcgaggcgcggcgagccgcagccattgccttttatggtaatcgtgcgagagggcgcagggacttcctttgtcccaaatctgtgcggagccgaaatctgggaggcgccgccgcaccccctctagcgggcgcggggcgaagcggtgcggcgccggcaggaaggaaatgggcggggagggccttcgtgcgtcgccgcgccgccgtccccttctccctctccagcctcggggctgtccgcggggggacggctgccttcgggggggacggggcagggcggggttcggcttctggcgtgtgaccggcggctctagagcctctgctaaccatgttcatgccttcttctttttcctacagctcctgggcaacgtgctggttattgtgctgtctcatcattttggcaaagaattg

SEQ ID NO: 24 - DNA, 522 bp, Artificial Sequence
  source: /note="Description of Artificial Sequence: Synthetic polynucleotide"
tcctcaggtgcaggctgcctatcagaaggtggtggctggtgtggccaatgccctggctcacaaataccactgagatctttttccctctgccaaaaattatggggacatcatgaagccccttgagcatctgacttctggctaataaaggaaatttattttcattgcaatagtgtgttggaattttttgtgtctctcactcggaaggacatatgggagggcaaatcatttaaaacatcagaatgagtatttggtttagagtttggcaacatatgcccatatgctggctgccatgaacaaaggttggctataaagaggtcatcagtatatgaaacagccccctgctgtccattccttattccatagaaaagccttgacttgaggttagattttttttatattttgttttgtgttatttttttctttaacatccctaaaattttccttacatgttttactagccagatttttcctcctctcctgactactcccagtcatagctgtccctcttctcttatggagatc

SEQ ID NO: 25 - DNA, 235 bp, Artificial Sequence
  source: /note="Description of Artificial Sequence: Synthetic polynucleotide"
ttaaccctagaaagataatcatattgtgacgtacgttaaagataatcatgcgtaaaattgacgcatgtgttttatcggtctgtatatcgaggtttatttattaatttgaatagatattaagttttattatatttacacttacatactaataataaattcaacaaacaatttatttatgtttatttatttattaaaaaaaaacaaaaactcaaaatttcttctataaagtaacaaa

SEQ ID NO: 26 - DNA, 6164 bp, Artificial Sequence
  source: /note="Description of Artificial Sequence: Synthetic polynucleotide"
ttaaccctagaaagatagtctgcgtaaaattgacgcatgcattcttgaaatattgctctctctttctaaatagcgcgaatccgtcgctgtgcatttaggacatctcagtcgccgcttggagctcccgtgaggcgtgcttgtcaatgcggtaagtgtcactgattttgaactataacgaccgcgtgagtcaaaatgacgcatgattatcttttacgtgacttttaagatttaactcatacgataattatattgttatttcatgttctacttacgtgataacttattatatatatattttcttgttatagatatcatcaactttgtatagaaaagttgctcgacattgattattgactagttattaatagtaatcaattacggggtcattagttcatagcccatatatggagttccgcgttacataacttacggtaaatggcccgcctggctgaccgcccaacgacccccgcccattgacgtcaataatgacgtatgttcccatagtaacgccaatagggactttccattgacgtcaatgggtggagtatttacggtaaactgcccacttggcagtacatcaagtgtatcatatgccaagtacgccccctattgacgtcaatgacggtaaatggcccgcctggcattatgcccagtacatgaccttatgggactttcctacttggcagtacatctacgtattagtcatcgctattaccatggtcgaggtgagccccacgttctgcttcactctccccatctcccccccctccccacccccaattttgtatttatttattttttaattattttgtgcagcgatgggggcggggggggggggggggcgcgcgccaggcggggcggggcggggcgaggggcggggcggggcgaggcggagaggtgcggcggcagccaatcagagcggcgcgctccgaaagtttccttttatggcgaggcggcggcggcggcggccctataaaaagcgaagcgcgcggcgggcgggagtcgctgcgcgctgccttcgccccgtgccccgctccgccgccgcctcgcgccgcccgccccggctctgactgaccgcgttactcccacaggtgagcgggcgggacggcccttctcctccgggctgtaattagcgcttggtttaatgacggcttgtttcttttctgtggctgcgtgaaagccttgaggggctccgggagggccctttgtgcggggggagcggctcggggggtgcgtgcgtgtgtgtgtgcgtggggagcgccgcgtgcggctccgcgctgcccggcggctgtgagcgctgcgggcgcggcgcggggctttgtgcgctccgcagtgtgcgcgaggggagcgcggccgggggcggtgccccgcggtgcggggggggctgcgaggggaacaaaggctgcgtgcggggtgtgtgcgtgggggggtgagcagggggtgtgggcgcgtcggtcgggctgcaaccccccctgcacccccctccccgagttgctgagcacggcccggcttcgggtgcggggctccgtacggggcgtggcgcggggctcgccgtgccgggcggggggtggcggcaggtgggggtgccgggcggggcggggccgcctcgggccggggagggctcgggggaggggcgcggcggcccccggagcgccggcggctgtcgaggcgcggcgagccgcagccattgccttttatggtaatcgtgcgagagggcgcagggacttcctttgtcccaaatctgtgcggagccgaaatctgggaggcgccgccgcaccccctctagcgggcgcggggcgaagcggtgcggcgccggcaggaaggaaatgggcggggagggccttcgtgcgtcgccgcgccgccgtccccttctccctctccagcctcggggctgtccgcggggggacggctgccttcgggggggacggggcagggcggggttcggcttctggcgtgtgaccggcggctctagagcctctgctaaccatgttcatgccttcttctttttcctacagctcctgggcaacgtgctggttattgtgctgtctcatcattttggcaaagaattgcaagtttgtacaaaaaagcaggctgccaccgaattcgcggccgctaaacccagctttcttgtacaaagtggcaactttattatacatagttgatcctcaggtgcaggctgcctatcagaaggtggtggctggtgtggccaatgccctggctcacaaataccactgagatctttttccctctgccaaaaattatggggacatcatgaagccccttgagcatctgacttctggctaataaaggaaatttattttcattgcaatagtgtgttggaattttttgtgtctctcactcggaaggacatatgggagggcaaatcatttaaaacatcagaatgagtatttggtttagagtttggcaacatatgcccatatgctggctgccatgaacaaaggttggctataaagaggtcatcagtatatgaaacagccccctgctgtccattccttattccatagaaaagccttgacttgaggttagattttttttatattttgttttgtgttatttttttctttaacatccctaaaattttccttacatgttttactagccagatttttcctcctctcctgactactcccagtcatagctgtccctcttctcttatggagatccctcgacctgcagcccaagcttggatccctcgagttaattaacgagagcataatattgatatgtgccaaagttgtttctgactgactaataagtataatttgtttctattatgtataggttaagctaattacttattttataatacaacatgactgtttttaaagtacaaaataagtttatttttgtaaaagagagaatgtttaaaagttttgttactttatagaagaaattttgagtttttgtttttttttaataaataaataaacataaataaattgtttgttgaatttattattagtatgtaagtgtaaatataataaaacttaatatctattcaaattaataaataaacctcgatatacagaccgataaaacacatgcgtcaattttacgcatgattatctttaacgtacgtcacaatatgattatctttctagggttaaataatagtttctaatttttttattattcagcctgctgtcgtgaataccgagctccaattcgccctatagtgagtcgtattacaattcactggccgtcgttttacaacgtcgtgactgggaaaaccctggcgttacccaacttaatcgccttgcagcacatccccctttcgccagctggcgtaatagcgaagaggcccgcaccgatcgcccttcccaacagttgcgcagcctgaatggcgaatgggacgcgccctgtagcggcgcattaagcgcggcgggtgtggtggttacgcgcagcgtgaccgctacacttgccagcgccctagcgcccgctcctttcgctttcttcccttcctttctcgccacgttcgccggctttccccgtcaagctctaaatcgggggctccctttagggttccgatttagtgctttacggcacctcgaccccaaaaaacttgattagggtgatggttcacgtagtgggccatcgccctgatagacggtttttcgccctttgacgttggagtccacgttctttaatagtggactcttgttccaaactggaacaacactcaaccctatctcggtctattcttttgatttataagggattttgccgatttcggcctattggttaaaaaatgagctgatttaacaaaaatttaacgcgaattttaacaaaatattaacgcttacaatttaggtggcacttttcggggaaatgtgcgcggaacccctatttgtttatttttctaaatacattcaaatatgtatccgctcatgagacaataaccctgataaatgcttcaataatattgaaaaaggaagagtatgagtattcaacatttccgtgtcgcccttattcccttttttgcggcattttgccttcctgtttttgctcacccagaaacgctggtgaaagtaaaagatgctgaagatcagttgggtgcacgagtgggttacatcgaactggatctcaacagcggtaagatccttgagagttttcgccccgaagaacgttttccaatgatgagcacttttaaagttctgctatgtggcgcggtattatcccgtattgacgccgggcaagagcaactcggtcgccgcatacactattctcagaatgacttggttgagtactcaccagtcacagaaaagcatcttacggatggcatgacagtaagagaattatgcagtgctgccataaccatgagtgataacactgcggccaacttacttctgacaacgatcggaggaccgaaggagctaaccgcttttttgcacaacatgggggatcatgtaactcgccttgatcgttgggaaccggagctgaatgaagccataccaaacgacgagcgtgacaccacgatgcctgtagcaatggcaacaacgttgcgcaaactattaactggcgaactacttactctagcttcccggcaacaattaatagactggatggaggcggataaagttgcaggaccacttctgcgctcggcccttccggctggctggtttattgctgataaatctggagccggtgagcgtgggtctcgcggtatcattgcagcactggggccagatggtaagccctcccgtatcgtagttatctacacgacggggagtcaggcaactatggatgaacgaaatagacagatcgctgagataggtgcctcactgattaagcattggtaactgtcagaccaagtttactcatatatactttagattgatttaaaacttcatttttaatttaaaaggatctaggtgaagatcctttttgataatctcatgaccaaaatcccttaacgtgagttttcgttccactgagcgtcagaccccgtagaaaagatcaaaggatcttcttgagatcctttttttctgcgcgtaatctgctgcttgcaaacaaaaaaaccaccgctaccagcggtggtttgtttgccggatcaagagctaccaactctttttccgaaggtaactggcttcagcagagcgcagataccaaatactgttcttctagtgtagccgtagttaggccaccacttcaagaactctgtagcaccgcctacatacctcgctctgctaatcctgttaccagtggctgctgccagtggcgataagtcgtgtcttaccgggttggactcaagacgatagttaccggataaggcgcagcggtcgggctgaacggggggttcgtgcacacagcccagcttggagcgaacgacctacaccgaactgagatacctacagcgtgagctatgagaaagcgccacgcttcccgaagagagaaaggcggacaggtatccggtaagcggcagggtcggaacaggagagcgcacgagggagcttccagggggaaacgcctggtatctttatagtcctgtcgggtttcgccacctctgacttgagcgtcgatttttgtgatgctcgtcaggggggcggagcctatggaaaaacgccagcaacgcggcctttttacggttcctggccttttgctggccttttgctcacatgttctttcctgcgttatcccctgattctgtggataaccgtattaccgcctttgagtgagctgataccgctcgccgcagccgaacgaccgagcgcagcgagtcagtgagcgaggaagcggaagagcgcccaatacgcaaaccgcctctccccgcgcgttggccgattcattaatgcagctggcacgacaggtttcccgactggaaagcgggcagtgagcgcaacgcaattaatgtgagttagctcactcattaggcaccccaggctttacactttatgcttccggctcgtatgttgtgtggaattgtgagcggataacaatttcacacaggaaacagctatgaccatgattacgccaagctcgaaattaaccctcactaaagggaacaaaagctggtacctcgcgcgacttggtttgccattctttagcgcgcgtcgcgtcacacagcttggccacaatgtggtttttgtcaaacgaagattctatgacgtgtttaaagtttaggtcgagtaaagcgcaaatctttt

SEQ ID NO: 27 - DNA, 6721 bp, Artificial Sequence
  source: /note="Description of Artificial Sequence: Synthetic polynucleotide"
ctcgacattgattattgactagttattaatagtaatcaattacggggtcattagttcatagcccatatatggagttccgcgttacataacttacggtaaatggcccgcctggctgaccgcccaacgacccccgcccattgacgtcaataatgacgtatgttcccatagtaacgccaatagggactttccattgacgtcaatgggtggagtatttacggtaaactgcccacttggcagtacatcaagtgtatcatatgccaagtacgccccctattgacgtcaatgacggtaaatggcccgcctggcattatgcccagtacatgaccttatgggactttcctacttggcagtacatctacgtattagtcatcgctattaccatggtcgaggtgagccccacgttctgcttcactctccccatctcccccccctccccacccccaattttgtatttatttattttttaattattttgtgcagcgatgggggcggggggggggggggggcgcgcgccaggcggggcggggcggggcgaggggcggggcggggcgaggcggagaggtgcggcggcagccaatcagagcggcgcgctccgaaagtttccttttatggcgaggcggcggcggcggcggccctataaaaagcgaagcgcgcggcgggcgggagtcgctgcgcgctgccttcgccccgtgccccgctccgccgccgcctcgcgccgcccgccccggctctgactgaccgcgttactcccacaggtgagcgggcgggacggcccttctcctccgggctgtaattagcgcttggtttaatgacggcttgtttcttttctgtggctgcgtgaaagccttgaggggctccgggagggccctttgtgcggggggagcggctcggggggtgcgtgcgtgtgtgtgtgcgtggggagcgccgcgtgcggctccgcgctgcccggcggctgtgagcgctgcgggcgcggcgcggggctttgtgcgctccgcagtgtgcgcgaggggagcgcggccgggggcggtgccccgcggtgcggggggggctgcgaggggaacaaaggctgcgtgcggggtgtgtgcgtgggggggtgagcagggggtgtgggcgcgtcggtcgggctgcaaccccccctgcacccccctccccgagttgctgagcacggcccggcttcgggtgcggggctccgtacggggcgtggcgcggggctcgccgtgccgggcggggggtggcggcaggtgggggtgccgggcggggcggggccgcctcgggccggggagggctcgggggaggggcgcggcggcccccggagcgccggcggctgtcgaggcgcggcgagccgcagccattgccttttatggtaatcgtgcgagagggcgcagggacttcctttgtcccaaatctgtgcggagccgaaatctgggaggcgccgccgcaccccctctagcgggcgcggggcgaagcggtgcggcgccggcaggaaggaaatgggcggggagggccttcgtgcgtcgccgcgccgccgtccccttctccctctccagcctcggggctgtccgcggggggacggctgccttcgggggggacggggcagggcggggttcggcttctggcgtgtgaccggcggctctagagcctctgctaaccatgttcatgccttcttctttttcctacagctcctgggcaacgtgctggttattgtgctgtctcatcattttggcaaagaattgcaagtttgtacaaaaaagcaggctgccaccatgcagattgagctgagcacctgtttcttcctgtgcctgctgagattttgcttctcagctacccgcaggtactacctgggagccgttgagctgtcctgggattacatgcagtcagatctgggggagctgcctgtggacgctcggtttccccccagagtgccaaagtcctttcccttcaacaccagcgtggtgtacaaaaagacactttttgttgaatttactgaccacttgttcaacatcgccaagccacgacccccatggatgggcctgctggggccaaccattcaggcagaggtttacgacacagtcgtgatcacactgaagaacatggcctcccatccagtgtctctgcacgccgtcggtgtgtcctactggaaagcatccgagggcgccgagtatgacgaccagaccagccagagagagaaagaggacgacaaagtgttccctggaggcagccacacctacgtgtggcaggtgttgaaggaaaatgggcccatggccagtgaccctttgtgtctgacttactcatacctgtctcatgtggatctagtcaaggacctgaattctggactgattggggcactgcttgtgtgccgcgaaggcagcctggccaaagaaaagacacagacccttcacaagttcatcctgctgttcgccgtgttcgacgaaggcaaatcctggcactcagaaaccaaaaactcactgatgcaggaccgggatgccgcctctgcccgcgcatggccaaaaatgcacaccgtcaacggctatgtcaatagaagtttgcccggcctcattggatgtcacaggaaaagcgtctattggcatgtaatcgggatgggaaccacacctgaggtccacagcatatttctggaaggccacacatttctggtgagaaatcatcgccaggcttccctggaaatttcccccatcaccttcttgaccgcccagacactgctcatggatcttgggcagtttctgctgttttgtcatatttcttctcaccaacacgacggaatggaggcctacgttaaggtcgatagttgccctgaagaacctcagctgaggatgaagaacaacgaggaagccgaggactacgatgacgatttgaccgattccgaaatggacgtggtgcgctttgatgatgacaattctccatccttcattcagattagatccgtcgccaagaagcaccccaagacctgggtgcactacattgcagccgaggaggaggattgggactacgcccccctggtgctggcacccgacgaccgaagctacaaatctcagtacctgaacaatggtccacaacggatcggcaggaagtacaagaaagtgcggttcatggcctatacagacgaaaccttcaaaaccagggaggctatccagcacgagtctgggattctgggaccactcctgtacggcgaagtgggcgacaccttgttaattatcttcaagaaccaggctagtagaccttataacatttatccccacggcattaccgatgtgcggcctctctactctaggcggcttccaaagggggtgaaacacctgaaggactttcccatcctccctggcgaaatctttaagtataagtggacagtgaccgtggaggatggaccaaccaagagcgaccccaggtgcctgacacgctattattcaagcttcgtgaatatggaaagggacctcgcatctggcttgatcggccctctgctgatatgttacaaggaaagcgtcgatcagagaggaaatcagatcatgtcagacaaaaggaatgtgatcctgttctccgtcttcgatgaaaacaggagctggtatctgacagagaacatccagagattcctgccaaatcccgccggcgtccagctggaggacccggagtttcaggcatctaacatcatgcattccattaatggttacgtgttcgactccctgcagctgagcgtgtgcctccacgaggtggcctactggtacatcttgagcatcggcgcccagaccgactttctgagcgtctttttctccgggtatactttcaaacataagatggtgtacgaagatactctgacgctgttccctttctctggggagactgtgtttatgtctatggagaaccctggactgtggattctcggatgccacaacagtgactttcgtaatagagggatgactgcactgctgaaggtgtccagctgtgataaaaatactggcgactactacgaagatagctatgaggatatctcagcatacctgctgagcaagaataacgccatcgagccccgaagcttctcacagaatccccctgtcctcaaggcccaccaggcggagatcacaaggaccacactccagtccgaccaggaggagattgactacgatgacacgatttctgtggagatgaaaaaagaggactttgacatctacgatgaggatgaaaaccagagccctaggtcgttccagaagaaaacaaggcactacttcattgccgccgtggagagactgtgggactacggaatgagtagttccccacacgtgttgcggaacagagcccagagtgggtccgtcccacagttcaagaaggttgttttccaggagttcacagatggctccttcactcagccactgtatcgcggcgagctgaatgagcacttgggcttattgggcccctacattcgcgcagaagtcgaagataatattatggtgaccttccgcaaccaggccagccggccttactcattctactcctctctcatctcttatgaggaggatcagcgccagggcgccgaaccccggaagaactttgtgaagcccaatgaaaccaaaacttacttttggaaggtgcagcaccatatggcgccgacgaaagacgaatttgactgcaaagcctgggcctacttcagcgacgtcgacttggagaaggacgtccacagcggcctgattggccctttgttggtctgccataccaatacactcaaccctgcccacgggaggcaggtgaccgtgcaggagtttgccttgttcttcaccatcttcgacgaaaccaagagctggtacttcacagagaacatggagaggaactgcagagcaccctgtaacatccagatggaggaccctactttcaaggaaaattacaggttccatgccattaatggctacatcatggataccctccccgggcttgtgatggctcaggaccagcgcatccgctggtacctgctctcaatgggctccaacgagaacattcatagcatccactttagtggccacgtgtttaccgtgcgcaagaaggaggagtacaagatggcactgtacaacctgtaccctggcgtgtttgagacagtggagatgctgccatccaaggccggcatctggcgcgtggagtgcctcattggggagcacctccatgctggcatgtctacactgttcctggtgtacagcaacaagtgtcagactccactcggaatggcctccgggcatatccgcgattttcagatcacggcctctggccagtatggccaatgggctcccaagctggccaggctgcactacagtgggagtatcaacgcttggagcaccaaggagcctttctcctggatcaaggtggacctgcttgcccccatgattattcacggcattaagacacagggggccaggcagaaattctcctccctgtacatctcccagttcatcatcatgtacagtctggacggcaaaaagtggcagacctaccgcgggaacagtaccgggacattgatggtgttcttcgggaacgtggactctagcggcattaaacacaacattttcaacccccccatcattgctaggtatatcaggctccatcccacccactatagcatcaggtccactctgcggatggagctgatgggctgcgaccttaattcatgcagcatgccgctgggcatggagtcaaaggccatctccgacgcccaaatcaccgcctccagctacttcaccaatatgttcgccacctggagccccagcaaggcccggctgcacctgcagggccgcagcaacgcctggcggcctcaggtgaacaaccccaaggagtggctgcaggtggacttccagaaaaccatgaaggtgactggggtcaccacccagggagtcaagagcctgctgaccagcatgtatgtgaaggagttcttgatcagctcgtcacaggatggccaccagtggactttgttctttcagaacggtaaggtgaaagtgttccagggaaaccaagattcctttacaccagtggtcaactctctggatcctcccctgctgacacggtacctgcggatccatccccagtcatgggtgcaccagattgctctgcgcatggaggtgcttggctgcgaggcccaggacctgtactgaaattcgcggccgctaaacccagctttcttgtacaaagtggcaactttattatacatagttgatcctcaggtgcaggctgcctatcagaaggtggtggctggtgtggccaatgccctggctcacaaataccactgagatctttttccctctgccaaaaattatggggacatcatgaagccccttgagcatctgacttctggctaataaaggaaatttattttcattgcaatagtgtgttggaattttttgtgtctctcactcggaaggacatatgggagggcaaatcatttaaaacatcagaatgagtatttggtttagagtttggcaacatatgcccatatgctggctgccatgaacaaaggttggctataaagaggtcatcagtatatgaaacagccccctgctgtccattccttattccatagaaaagccttgacttgaggttagattttttttatattttgttttgtgttatttttttctttaacatccctaaaattttccttacatgttttactagccagatttttcctcctctcctgactactcccagtcatagctgtccctcttctcttatggagatc

SEQ ID NO: 28 - DNA, 3733 bp, Artificial Sequence
  source: /note="Description of Artificial Sequence: Synthetic polynucleotide"
ctcgacattgattattgactagttattaatagtaatcaattacggggtcattagttcatagcccatatatggagttccgcgttacataacttacggtaaatggcccgcctggctgaccgcccaacgacccccgcccattgacgtcaataatgacgtatgttcccatagtaacgccaatagggactttccattgacgtcaatgggtggagtatttacggtaaactgcccacttggcagtacatcaagtgtatcatatgccaagtacgccccctattgacgtcaatgacggtaaatggcccgcctggcattatgcccagtacatgaccttatgggactttcctacttggcagtacatctacgtattagtcatcgctattaccatggtcgaggtgagccccacgttctgcttcactctccccatctcccccccctccccacccccaattttgtatttatttattttttaattattttgtgcagcgatgggggcggggggggggggggggcgcgcgccaggcggggcggggcggggcgaggggcggggcggggcgaggcggagaggtgcggcggcagccaatcagagcggcgcgctccgaaagtttccttttatggcgaggcggcggcggcggcggccctataaaaagcgaagcgcgcggcgggcgggagtcgctgcgcgctgccttcgccccgtgccccgctccgccgccgcctcgcgccgcccgccccggctctgactgaccgcgttactcccacaggtgagcgggcgggacggcccttctcctccgggctgtaattagcgcttggtttaatgacggcttgtttcttttctgtggctgcgtgaaagccttgaggggctccgggagggccctttgtgcggggggagcggctcggggggtgcgtgcgtgtgtgtgtgcgtggggagcgccgcgtgcggctccgcgctgcccggcggctgtgagcgctgcgggcgcggcgcggggctttgtgcgctccgcagtgtgcgcgaggggagcgcggccgggggcggtgccccgcggtgcggggggggctgcgaggggaacaaaggctgcgtgcggggtgtgtgcgtgggggggtgagcagggggtgtgggcgcgtcggtcgggctgcaaccccccctgcacccccctccccgagttgctgagcacggcccggcttcgggtgcggggctccgtacggggcgtggcgcggggctcgccgtgccgggcggggggtggcggcaggtgggggtgccgggcggggcggggccgcctcgggccggggagggctcgggggaggggcgcggcggcccccggagcgccggcggctgtcgaggcgcggcgagccgcagccattgccttttatggtaatcgtgcgagagggcgcagggacttcctttgtcccaaatctgtgcggagccgaaatctgggaggcgccgccgcaccccctctagcgggcgcggggcgaagcggtgcggcgccggcaggaaggaaatgggcggggagggccttcgtgcgtcgccgcgccgccgtccccttctccctctccagcctcggggctgtccgcggggggacggctgccttcgggggggacggggcagggcggggttcggcttctggcgtgtgaccggcggctctagagcctctgctaaccatgttcatgccttcttctttttcctacagctcctgggcaacgtgctggttattgtgctgtctcatcattttggcaaagaattgcaagtttgtacaaaaaagcaggctgccaccatgcagcgcgtgaacatgattatggccgagtctcccggcctgatcaccatctgtctgctgggctatctgctgagcgccgagtgcaccgtgtttctggatcacgagaacgccaacaagatcctgaacagacccaagcggtacaacagcggcaagctggaagagttcgtgcagggcaacctggaacgcgagtgcatggaagagaagtgcagcttcgaagaggccagagaggtgttcgagaacaccgagagaaccaccgagttctggaagcagtacgtggacggcgatcagtgcgagagcaacccttgtctgaatggcggcagctgcaaggacgacatcaacagctacgagtgctggtgccccttcggcttcgagggcaagaattgcgagctggacgtgacctgcaacatcaagaacggcagatgcgagcagttctgcaagaacagcgccgacaacaaggtcgtgtgctcctgcacagagggctacagactggccgagaaccagaagtcttgcgagcccgctgtgccctttccatgtggcagagtgtctgtgtcccagaccagcaagctgaccagagccgagacagtgttccccgacgtggactacgtgaacagcaccgaggccgagacaatcctggacaacatcacccagagcacccagtccttcaacgacttcaccagagtcgtcggcggcgaggatgctaagcctggacagtttccttggcaagtggtgctgaacggcaaggtggacgctttttgtggcggctccatcgtgaacgagaagtggatcgtgaccgccgctcactgtgtggaaaccggcgtgaagattacagtggtggccggcgagcacaacatcgaggaaacagagcacaccgagcagaaacggaacgtgatcagaatcatccctcaccacaactacaacgccgccatcaacaagtacaaccacgatatcgccctgctggaactggacgagcccctggtcctgaactcttacgtgacccctatctgtatcgccgacaaagagtacaccaacatctttctgaagttcggcagcggctacgtgtccggctggggaagagttttccacaagggcagatcagccctggtgctgcagtacctgagagtgcccctggtggatagagccacatgcctgctgagcaccaagttcaccatctacaacaacatgttctgcgccggcttccacgaaggcggcagagattcttgtcaaggcgattctggcggccctcacgtgacagaggttgagggcacaagctttctgaccggcatcatcagctggggcgaagagtgtgccatgaaggggaagtacggcatctacaccaaggtgtccagatacgtgaactggatcaaagaaaagaccaagctcacctgaaattcgcggccgctaaacccagctttcttgtacaaagtggcaactttattatacatagttgatcctcaggtgcaggctgcctatcagaaggtggtggctggtgtggccaatgccctggctcacaaataccactgagatctttttccctctgccaaaaattatggggacatcatgaagccccttgagcatctgacttctggctaataaaggaaatttattttcattgcaatagtgtgttggaattttttgtgtctctcactcggaaggacatatgggagggcaaatcatttaaaacatcagaatgagtatttggtttagagtttggcaacatatgcccatatgctggctgccatgaacaaaggttggctataaagaggtcatcagtatatgaaacagccccctgctgtccattccttattccatagaaaagccttgacttgaggttagattttttttatattttgttttgtgttatttttttctttaacatccctaaaattttccttacatgttttactagccagatttttcctcctctcctgactactcccagtcatagctgtccctcttctcttatggagatc

SEQ ID NO: 29 - protein, 153 aa, Artificial Sequence
  source: /note="Description of Artificial Sequence: Synthetic polypeptide"
MYRMQLLSCIALSLALVTNSAPTSSSTKKTQLQLEHLLLDLQMILNGINNYKNPKLTRMLTFKFYMPKKATELKHLQCLEEELKPLEEVLNLAQSKNFHLRPRDLISNINVIVLELKGSETTFMCEYADETATIVEFLNRWITFCQSIISTLT

SEQ ID NO: 30 - protein, 65 aa, Artificial Sequence
  source: /note="Description of Artificial Sequence: Synthetic polypeptide"
MIPAKDMAKVMIVMLAICFLTKSDGKSVKKRSVSEIQLMHNLGKHLNSMERVEWLRKKLQDVHNF

SEQ ID NO: 31 - protein, 115 aa, Artificial Sequence
  source: /note="Description of Artificial Sequence: Synthetic polypeptide"
MIPAKDMAKVMIVMLAICFLTKSDGKSVKKRSVSEIQLMHNLGKHLNSMERVEWLRKKLQDVHNFVALGAPLAPRDAGSQRPRKKEDNVLVESHEKSLGEADKADVNVLTKAKSQ

SEQ ID NO: 32 - protein, 506 aa, Artificial Sequence
  source: /note="Description of Artificial Sequence: Synthetic polypeptide"
MIPARFAGVLLALALILPGTLCSLSCRPPMVKLVCPADNLRAEGLECTKTCQNYDLECMSMGCVSGCLCPPGMVRHENRCVALERCPCFHQGKEYAPGETVKIGCNTCVCRDRKWNCTDHVCDATCSTIGMAHYLTFDGLKYLFPGECQYVLVQDYCGSNPGTFRILVGNKGCSHPSVKCKKRVTILVEGGEIELFDGEVNVKRPMKDETHFEVVESGRYIILLLGKALSVVWDRHLSISVVLKQTYQEKVCGLCGNFDGIQNNDLTSSNLQVEEDPVDFGNSWKVSSQCADTRKVPLDSSPATCHNNIMKQTMVDSSCRILTSDVFQDCNKLVDPEPYLDVCIYDTCSCESIGDCACFCDTIAAYAHVCAQHGKVVTWRTATLCPQSCEERNLRENGYECEWRYNSCAPACQVTCQHPEPLACPVQCVEGCHAHCPPGKILDELLQTCVDPEDCPVCEVAGRRFASGKKVTLNPSDPEHCQICHCDVVNLTCEACQEPGGLVVPP

SEQ ID NO: 33 - protein, 1247 aa, Artificial Sequence
  source: /note="Description of Artificial Sequence: Synthetic polypeptide"
MIPARFAGVLLALALILPGTLCAEGTRGRSSTARCSLFGSDFVNTFDGSMYSFAGYCSYLLAGGCQKRSFSIIGDFQNGKRVSLSVYLGEFFDIHLFVNGTVTQGDQRVSMPYASKGLYLETEAGYYKLSGEAYGFVARIDGSGNFQVLLSDRYFNKTCGLCGNFNIFAEDDFMTQEGTLTSDPYDFANSWALSSGEQWCERASPPSSSCNISSGEMQKGLWEQCQLLKSTSVFARCHPLVDPEPFVALCEKTLCECAGGLECACPALLEYARTCAQEGMVLYGWTDHSACSPVCPAGMEYRQCVSPCARTCQSLHINEMCQERCVDGCSCPEGQLLDEGLCVESTECPCVHSGKRYPPGTSLSRDCNTCICRNSQWICSNEECPGECLVTGQSHFKSFDNRYFTFSGICQYLLARDCQDHSFSIVIETVQCADDRDAVCTRSVTVRLPGLHNSLVKLKHGAGVAMDGQDVQLPLLKGDLRIQHTVTASVRLSYGEDLQMDWDGRGRLLVKLSPVYAGKTCGLCGNYNGNQGDDFLTPSGLAEPRVEDFGNAWKLHGDCQDLQKQHSDPCALNPRMTRFSEEACAVLTSPTFEACHRAVSPLPYLRNCRYDVCSCSDGRECLCGALASYAAACAGRGVRVAWREPGRCELNCPKGQVYLQCGTPCNLTCRSLSYPDEECNEACLEGCFCPPGLYMDERGDCVPKAQCPCYYDGEIFQPEDIFSDHHTMCYCEDGFMHCTMSGVPGSLLPDAVLSSPLSHRSKRSLSCRPPMVKLVCPADNLRAEGLECTKTCQNYDLECMSMGCVSGCLCPPGMVRHENRCVALERCPCFHQGKEYAPGETVKIGCNTCVCRDRKWNCTDHVCDATCSTIGMAHYLTFDGLKYLFPGECQYVLVQDYCGSNPGTFRILVGNKGCSHPSVKCKKRVTILVEGGEIELFDGEVNVKRPMKDETHFEVVESGRYIILLLGKALSVVWDRHLSISVVLKQTYQEKVCGLCGNFDGIQNNDLTSSNLQVEEDPVDFGNSWKVSSQCADTRKVPLDSSPATCHNNIMKQTMVDSSCRILTSDVFQDCNKLVDPEPYLDVCIYDTCSCESIGDCACFCDTIAAYAHVCAQHGKVVTWRTATLCPQSCEERNLRENGYECEWRYNSCAPACQVTCQHPEPLACPVQCVEGCHAHCPPGKILDELLQTCVDPEDCPVCEVAGRRFASGKKVTLNPSDPEHCQICHCDVVNLTCEACQEPGGLVVPP

SEQ ID NO: 34 - protein, 232 aa, Artificial Sequence
  source: /note="Description of Artificial Sequence: Synthetic polypeptide"
EPKSCDKTHTCPPCPAPELLGGPSVFLFPPKPKDTLMISRTPEVTCVVVDVSHEDPEVKFNWYVDGVEVHNAKTKPREEQYNSTYRVVSVLTVLHQDWLNGKEYKCKVSNKALPAPIEKTISKAKGQPREPQVYTLPPSRDELTKNQVSLTCLVKGFYPSDIAVEWESNGQPENNYKTTPPVLDSDGSFFLYSKLTVDKSRWQQGNVFSCSVMHEALHNHYTQKSLSLSPGK

SEQ ID NO: 35 - protein, 585 aa, Artificial Sequence [sequence omitted]

SEQ ID NO: 36 - protein, 461 aa, Artificial Sequence
  source: /note="Description of Artificial Sequence: Synthetic polypeptide"
MQRVNMIMAESPGLITICLLGYLLSAECTVFLDHENANKILNRPKRYNSGKLEEFVQGNLERECMEEKCSFEEAREVFENTERTTEFWKQYVDGDQCESNPCLNGGSCKDDINSYECWCPFGFEGKNCELDVTCNIKNGRCEQFCKNSADNKVVCSCTEGYRLAENQKSCEPAVPFPCGRVSVSQTSKLTRAETVFPDVDYVNSTEAETILDNITQSTQSFNDFTRVVGGEDAKPGQFPWQVVLNGKVDAFCGGSIVNEKWIVTAAHCVETGVKITVVAGEHNIEETEHTEQKRNVIRIIPHHNYNAAINKYNHDIALLELDEPLVLNSYVTPICIADKEYTNIFLKFGSGYVSGWGRVFHKGRSALVLQYLRVPLVDRATCLLSTKFTIYNNMFCAGFHEGGRDSCQGDSGGPHVTEVEGTSFLTGIISWGEECAMKGKYGIYTKVSRYVNWIKEKTKLT

SEQ ID NO: 37 - protein, 12 aa, Artificial Sequence
  source: /note="Description of Artificial Sequence: Synthetic peptide"
SWELYYPLRANL

SEQ ID NO: 38 - protein, 5 aa, Artificial Sequence
  source: /note="Description of Artificial Sequence: Synthetic peptide"
HAVDI

SEQ ID NO: 39 - protein, 4 aa, Artificial Sequence
  source: /note="Description of Artificial Sequence: Synthetic peptide"
DGEA

SEQ ID NO: 40 - protein, 6 aa, Artificial Sequence
  source: /note="Description of Artificial Sequence: Synthetic peptide"
FYFDLR

SEQ ID NO: 41 - protein, 6 aa, Artificial Sequence
  source: /note="Description of Artificial Sequence: Synthetic peptide"
  MOD_RES (3)..(3): 4-hydroxyproline
GFXGER

SEQ ID NO: 42 - protein, 4 aa, Artificial Sequence
  source: /note="Description of Artificial Sequence: Synthetic peptide"
VAPG

SEQ ID NO: 43 - protein, 3 aa, Artificial Sequence
  source: /note="Description of Artificial Sequence: Synthetic peptide"
RGD

SEQ ID NO: 44 - protein, 3 aa, Artificial Sequence
  source: /note="Description of Artificial Sequence: Synthetic peptide"
GPR

SEQ ID NO: 45 - protein, 6 aa, Artificial Sequence
  source: /note="Description of Artificial Sequence: Synthetic peptide"
KQAGDV

SEQ ID NO: 46 - protein, 5 aa, Artificial Sequence
  source: /note="Description of Artificial Sequence: Synthetic peptide"
PHSRN

SEQ ID NO: 47 - protein, 4 aa, Artificial Sequence
  source: /note="Description of Artificial Sequence: Synthetic peptide"
REDV

SEQ ID NO: 48 - protein, 5 aa, Artificial Sequence
  source: /note="Description of Artificial Sequence: Synthetic peptide"
IKVAV

SEQ ID NO: 49 - protein, 3 aa, Artificial Sequence
  source: /note="Description of Artificial Sequence: Synthetic peptide"
LRE

SEQ ID NO: 50 - protein, 5 aa, Artificial Sequence
  source: /note="Description of Artificial Sequence: Synthetic peptide"
YIGSR

SEQ ID NO: 51 - protein, 7 aa, Artificial Sequence
  source: /note="Description of Artificial Sequence: Synthetic peptide"
SVVYGLR

SEQ ID NO: 52 - protein, 8 aa, Artificial Sequence
  source: /note="Description of Artificial Sequence: Synthetic peptide"
AEIDGIEL

SEQ ID NO: 53 - protein, 4 aa, Artificial Sequence
  source: /note="Description of Artificial Sequence: Synthetic peptide"
VTCG

SEQ ID NO: 54 - protein, 37 aa, Artificial Sequence
  source: /note="Description of Artificial Sequence: Synthetic polypeptide"
  MOD_RES (19)..(19): 4-hydroxyproline
PGPPGPPGPPGPPGPPGFXGERGPPGPPGPPGPPGPP

SEQ ID NO: 55 - protein, 15 aa, Artificial Sequence
  source: /note="Description of Artificial Sequence: Synthetic peptide"
PHSRNGGGGGGRGDS

SEQ ID NO: 56 - protein, 17 aa, Artificial Sequence
  source: /note="Description of Artificial Sequence: Synthetic peptide"
SRARKQAASIKVAVADR

SEQ ID NO: 57 - protein, 6 aa, Artificial Sequence
  source: /note="Description of Artificial Sequence: Synthetic peptide"
KQLREQ

SEQ ID NO: 58 - protein, 5 aa, Artificial Sequence
  source: /note="Description of Artificial Sequence: Synthetic peptide"
SVTCG

SEQ ID NO: 59 - protein, 5 aa, Artificial Sequence
  source: /note="Description of Artificial Sequence: Synthetic peptide"
RGDSP

SEQ ID NO: 60 - protein, 6 aa, Artificial Sequence
  source: /note="Description of Artificial Sequence: Synthetic peptide"
GRGDSP

SEQ ID NO: 61 - protein, 4 aa, Artificial Sequence
  source: /note="Description of Artificial Sequence: Synthetic peptide"
GGGG

SEQ ID NO: 62 - protein, 4 aa, Artificial Sequence
  source: /note="Description of Artificial Sequence: Synthetic peptide"
GRGD

SEQ ID NO: 63 - protein, 6 aa, Artificial Sequence
  source: /note="Description of Artificial Sequence: Synthetic peptide"
  SITE (1)..(3): /note="This region may encompass 1-3 residues"
GGGRGD

SEQ ID NO: 64 - protein, 8 aa, Artificial Sequence
  source: /note="Description of Artificial Sequence: Synthetic peptide"
  SITE (1)..(3): /note="This region may encompass 1-3 residues"
GGGRGDSP

SEQ ID NO: 65 - protein, 6 aa, Artificial Sequence
  source: /note="Description of Artificial Sequence: Synthetic peptide"
LKRHQR

SEQ ID NO: 66 - protein, 7 aa, Artificial Sequence
  source: /note="Description of Artificial Sequence: Synthetic peptide"
  SITE (1)..(3): /note="This region may encompass 1-3 residues"
GGGDGEA

SEQ ID NO: 67 - protein, 8 aa, Artificial Sequence
  source: /note="Description of Artificial Sequence: Synthetic peptide"
  SITE (1)..(3): /note="This region may encompass 1-3 residues"
GGGPHRSN

SEQ ID NO: 68 - protein, 7 aa, Artificial Sequence
  source: /note="Description of Artificial Sequence: Synthetic peptide"
  SITE (1)..(3): /note="This region may encompass 1-3 residues"
GGGREDV

SEQ ID NO: 69 - protein, 6 aa, Artificial Sequence
  source: /note="Description of Artificial Sequence: Synthetic peptide"
GGGGGG

SEQ ID NO: 70 - protein, 4 aa, Artificial Sequence
  source: /note="Description of Artificial Sequence: Synthetic peptide"
  SITE (1)..(4): /note="This sequence may encompass 1-4 residues"
GGGG